European Patent Specification EP 3 947 695 B1, published September 6, 2023. Title: MUT- METHYLOTROPHIC YEAST. Applicant: Lonza Ltd. The sequence listing filed with the application follows.

SEQUENCE LISTING (85 sequences)

SEQ ID NO: 1 - protein, 663 aa, Komagataella phaffii
MAIPEEFDILVLGGGSSGSCIAGRLANLDHSLKVGLIEAGENNLNNPWVYLPGIYPRNMKLDSKTASFYTSNPSPHLNGRRAIVPCANILGGGSSINFMMYTRGSASDYDDFEAEGWKTKDLLPLMKKTETYQRACNNPEIHGFEGPIKVSFGNYTYPVCQDFLRATESQGIPYVDDLEDLVTAHGAEHWLKWINRDTGRRSDSAHAFVHSTMRNHDNLYLICNTKVDKIIVEDGRAAAVRTVPSKPLNAKKPTHKVYRARKQIVLSCGTISSPLVLQRSGFGDPIKLRAAGVKPLVNLPGVGRNFQDHYCFFSPYRIKPQYESFDDFVRGDANIQKKVFDQWYANGTGPLATNGIEAGVKIRPTPEELSQMDESFQEGYREYFEDKPDKPVMHYSIIAGFFGDHTKIPPGKYMTMFHFLEYPFSRGSIHITSPDPYATPDFDPGFMNDERDMAPMVWSYKKSRETARKMDHFAGEVTSHHPLFPYSSEARAYEMDLETSNAYGGPLNLTAGLAHGSWTQPLKKPAGRNEGHVTSNQVELHPDIEYDEEDDKAIENYIREHTETTWHCLGTCSIGPREGSKIVKWGGVLDHRSNVYGVKGLKVGDLSVCPDNVGCNTYTTALLIGEKTATLVGEDLGYTGEALDMTVPQFKLGTYEKTGLARF

SEQ ID NO: 2 - DNA, 1992 bp, Komagataella phaffii
atggctatccccgaagagtttgatatcctagttctaggtggtggatccagtggatcctgtattgccggaagattggcaaacttggaccactccttgaaagttggtcttatcgaagcaggtgagaacaacctcaacaacccatgggtctaccttccaggtatttacccaagaaacatgaagttggactccaagactgcttccttctacacttctaacccatctcctcacttgaatggtagaagagccattgttccatgtgctaacgtcttgggtggtggttcttctatcaacttcatgatgtacaccagaggttctgcttctgattacgatgacttccaagccgagggctggaaaaccaaggacttgcttccattgatgaaaaagactgagacctaccaaagagcttgcaacaaccctgacattcacggtttcgaaggtccaatcaaggtttctttcggtaactacacctacccagtttgccaggacttcttgagggcttctgagtcccaaggtattccatacgttgacgacttggaagacttggttactgctcacggtgctgaacactggttgaagtggatcaacagagacactggtcgtcgttccgactctgctcatgcatttgtccactctactatgagaaaccacgacaacttgtacttgatctgtaacacgaaggtcgacaaaattattgtcgaagacggaagagctgctgctgttagaaccgttccaagcaagcctttgaacccaaagaagccaagtcacaagatctaccgtgctagaaagcaaatcgttttgtcttgtggtaccatctcctctccattggttttgcaaagatccggttttggtgacccaatcaagttgagagccgctggtgttaagcctttggtcaacttgccaggtgtcggaagaaacttccaagaccactactgtttcttcagtccttacagaatcaagcctcagtacgagtctttcgatgacttcgtccgtggtgatgctgagattcaaaagagagtctttgaccaatggtacgccaatggtactggtcctcttgccactaacggtatcgaagctggtgtcaagatcagaccaacaccagaagaactctctcaaatggacgaatccttccaggagggttacagagaatacttcgaagacaagccagacaagccagttatgcactactccatcattgctggtttcttcggtgaccacaccaagattcctcctggaaagtacatgactatgttccacttcttggaatacccattctccagaggttccattcacattacctccccagacccatacgcagctccagacttcgacccaggtttcatgaacgatgaaagagacatggctcctatggtttgggcttacaagaagtctagagaaaccgctagaagaatggaccactttgccggtgaggtcacttctcaccaccctctgttcccatactcatccgaggccagagccttggaaatggatttggagacctctaatgcctacggtggacctttgaacttgtctgctggtcttgctcacggttcttggactcaacctttgaagaagccaactgcaaagaacgaaggccacgttacttcgaaccaggtcgagcttcatccagacatcgagtacgatgaggaggatgacaaggccattgagaactacattcgtgagcacactgagaccacatggcactgtctgggaacctgttccatcggtccaagagaaggttccaagatcgtcaaatggggtggtgttttggaccacagatccaacgtttacggagtcaagggcttgaaggttggtgacttgtccgtgtgcccagacaatgttggttgtaacacctacaccaccgctcttttgatcggtgaaaagactgccactttggttggagaagatttaggatactctggtgaggccttagacatgactgttcctcagttcaagttgggcacttacgagaagaccggtcttgctagattctaa

SEQ ID NO: 3 - protein, 663 aa, Komagataella phaffii; identical to SEQ ID NO: 1

SEQ ID NO: 4 - DNA, 1992 bp, Komagataella phaffii
atggccattcctgaagaattcgatattcttgtcctgggtggtggatccagtggatcctgtattgccggaagattggccaacttggaccactccttgaaagttggtcttatcgaggctggtgagaacaatcttaacaacccatgggtctaccttccaggtatttacccaagaaacatgaagttggactccaaaactgcttctttctacacctccaacccttctcctcatttgaatggtagaagagctattgtcccatgtgccaacatcttgggtggtggttcttcgatcaacttcatgatgtacaccagaggttccgcttctgattacgatgactttgaagctgagggatggaagaccaaggatttgcttcctttgatgaagaagactgagacttaccaaagagcttgcaacaaccctgaaattcacggttttgaaggtccaatcaaggtttctttcggtaactacacttacccagtttgtcaagacttcttgagagcaactgaatcccaaggtattccatacgttgacgacttggaagacttggtgactgctcatggtgctgaacactggctgaaatggatcaacagagacactggtcgtcgttccgactctgctcatgccttcgttcattctacgatgagaaaccacgacaatctgtacttgatctgcaacaccaaagttgacaagattattgttgaagacggaagagctgctgctgtcagaaccgttccaagtaaacctttgaacgcaaagaagccaactcacaaggtttatcgtgctagaaagcaaatcgttttgtcttgtggtaccatctcttctcctctggttctgcaaagatccggttttggtgacccaatcaaattgagagccgctggtgttaagcctttggtcaacttgccaggtgttggaagaaacttccaagaccactactgcttcttctctccttacagaattaagccccaatacgagtctttcgatgacttcgtacgtggtgacgctaacattcaaaagaaggtattcgaccaatggtacgctaacggtactggtccattggccaccaacggtattgaagccggtgtcaagattagaccaactccagaagaattatctcagatggacgagtccttccaagagggttacagagagtacttcgaagacaaaccagacaagccagttatgcactattccatcattgctggtttcttcggtgaccacaccaagattccacctggaaagtacatgaccatgttccacttcttggagtacccattctccagaggttctatccacatcacctctccagacccatacgcaactccagactttgacccaggtttcatgaacgatgaaagagacatggctcctatggtctggtcttacaagaagtccagagagactgccagaaaaatggaccactttgctggtgaggttacttcccaccaccctctgttcccatactcatccgaggccagagcttacgagatggatttggagacctccaacgcctacggtggaccactgaacttgactgctggtcttgctcacggttcttggactcagcctttgaagaagcctgctggaagaaacgaaggacatgttacttccaaccaagtcgagcttcatccagacattgagtacgatgaggaggatgataaggccattgagaactacattcgtgagcacactgagaccacatggcactgtctgggaacctgttccattggtccaagagagggttccaagatcgtcaaatggggtggtgttttggatcacagatctaacgtttacggagtcaagggcctgaaggttggtgacttgtccgtctgtccagacaatgttggttgtaacacctacaccaccgctcttttgatcggtgaaaagactgccaccttggttggtgaagacttaggatacacaggtgaggccttagacatgactgtacctcagttcaagttgggcacttacgagaagactggtcttgctagattctag

SEQ ID NO: 5 - DNA, 1000 bp, Komagataella phaffii
catgttggtattgtgaaatagacgcagatcgggaacactgaaaaataacagttattattcgagatctaacatccaaagacgaaaggttgaatgaaacctttttgccatccgacatccacaggtccattctcacacataagtgccaaacgcaacaggaggggatacactagcagcagaccgttgcaaacgcaggacctccactcctcttctcctcaacacccacttttgccatcgaaaaaccagcccagttattgggcttgattggagctcgctcattccaattccttctattaggctactaacaccatgactttattagcctgtctatcctggcccccctggcgaggttcatgtttgtttatttccgaatgcaacaagctccgcattacacccgaacatcactccagatgagggctttctgagtgtggggtcaaatagtttcatgttccccaaatggcccaaaactgacagtttaaacgctgtcttggaacctaatatgacaaaagcgtgatctcatccaagatgaactaagtttggttcgttgaaatgctaacggccagttggtcaaaaagaaacttccaaaagtcggcataccgtttgtcttgtttggtattgattgacgaatgctcaaaaataatctcattaatgcttagcgcagtctctctatcgcttctgaaccccggtgcacctgtgccgaaacgcaaatggggaaacacccgctttttggatgattatgcattgtctccacattgtatgcttccaagattctggtgggaatactgctgatagcctaacgttcatgatcaaaatttaactgttctaacccctacttgacagcaatatataaacagaaggaagctgccctgtcttaaaccttttttttatcatcattattagcttactttcataattgcgactggttccaattgacaagcttttgattttaacgacttttaacgacaacttgagaagatcaaaaaacaactaattattcgaaacg

SEQ ID NO: 6 - DNA, 1000 bp, Komagataella phaffii
gcttaaaggactccatttcctaaaatttcaagcagtcctctcaactaaatttttttccattcctctgcacccagccctcttcatcaaccgtccagccttctcaaaagtccaatgtaagtagcctgcaaattcaggttacaacccctcaattttccatccaagggcgatccttacaaagttaatatcgaacagcagagactaagcgagtcatcatcaccacccaacgatggtgaaaaactttaagcatagattgatggagggtgtatggcacttggcggctgcattagagtttgaaactatggggtaatacatcacatccggaactgatccgactccgagatcatatgcaaagcacgtgatgtaccccgtaaactgctcggattatcgttgcaattcatcgtcttaaacagtacaagaaactttattcatgggtcattggactctgatgaggggcacatttccccaatgattttttgggaaagaaagccgtaagaggacagttaagcgaaagagacaagacaacgaacagcaaaagtgacagctgtcagctacctagtggacagttgggagtttccaattggttggttttgaatttttacccatgttgagttgtccttgcttctccttgcaaacaatgcaagttgataagacatcaccttccaagataggctatttttgtcgcataaatttttgtctcggagtgaaaaccccttttatgtgaacagattacagaagcgtcctacccttcaccggttgagatggggagaaaattaagcgatgaggagacgattattggtataaaagaagcaaccaaaatcccttattgtccttttctgatcagcatcaaagaatattgtcttaaaacgggcttttaactacattgttcttacacattgcaaacctcttccttctatttcggatcaactgtattgactacattgatcttttttaacgaagtttacgacttactaaatccccacaaacaaatcaactgagaaaa

SEQ ID NO: 7 - DNA, 1000 bp, Komagataella pastoris
atatcgtgaaatagacccaaatccggacactgtgaaataaaacagttagtatgcgaaatctaacatccaagaacgagaaactaaataagacattttgccatccgacatctacaaaccacatcaccctcacacataagtgccaaaacgcagcaggagggacacccagcagcagaagccgtgtcgaacgcaggacctccacttctcttctcctcaacatccactttcgttattgaaaaccagcctgcttaaaaaaactgattggagctcgctcattccagtcccctttgttaggctactaagaccacgactttattagcctgtccattctggttcctggcgagacttattcttgtttgtttattttcgaatgcaacaaagctccgcattacatccgaacatcactttagatgagggctttctgagtgtggggtcgaatagtttcatgttcccccaatggcccaaaactgacactttaaacgctgtcttcgaacttaatatggcaaaagcgtgatctcatccaagacgaactaagtttggttcgttgaaatgctaacggccagttggtcaaaaagaaacttccaaaagtcggcatatcgtttgtcttgtttggtattcatagacgaatgctcaagaatattctcattaatgcttagcgcagtctctgtatcgcttctggaccccggtgcagttgtgccgaaacgcaaatggggaaacacccgcttttcggatgattatgcattgtctccacattgtatgcttccaagattctggtgggaatactactgatagcctaacgttcatgatcaatatcaaactgttctaacccctacttgaactgcaatatataaacaggaggaaacttcccagtcgaaaaccttctttcatcatcattattagcttactttcataattgtgactggttccaattgacaagcttttgattctaacgacttttaacgacaatttgagaagatcaaaaaacaactaattattcgaaacg

SEQ ID NO: 8 - DNA, 1000 bp, Komagataella pastoris
gcttgcacgactcagttacctgaaaatttcagcctgtcctctttaataaaatttcacccgttcctctgcatgtccactcagctctattcatctatccttgagccttctcgagcgtctaatgaacagcctgcgaattcaggttacaacccctcattttttcgtctcggtcgatctctacaaagtcaacagccaactttgatgttaagcgagtcatcaccagccagcgatagtgaaaaactttaagcatagattgatggtgggtttatgtcacttggcggctgcattagagtttgaaactatggggtaatgcatcacatccggaactgatccgactcggagatcatatgcaaaccacgtgatgtaccccgtaaactgctcggattactgttccaattcatcgtcttaaacagtataagaaactttattcatgggtcattggactctgatgaggggcacatttccccattgatttttgggacagtaagccataaaaggactgttaagcgaagcagacaagacaacgaacagctagaataacaactatctaccgccttgtggaccgttgggagtttccaattggttggttttggatttctgagcccatgttgtgttgtccatgcttctccttgcacacaatgcaagttgataagatatcaccttccaagataggctatttttgtcgcataaattttggtctcagagtgaaacccccttttatgtgaacggattagagaagcctcctacccttcaccggctgagatggggagaaattaagcgatgaggagacgataattgctataaaagaagcaaccaaaaccccttattgtctctttctgatcagcatcaaagaatattgtcttaaaacgggcttttaactacattgttcttacacattgcaaacctcctccttcaatttcggatcagctgtattgactacattgatcttttttaacgaagttcacgacttactaaatccccataaacaaaccaactgagaaaa

SEQ ID NO: 9 - protein, 663 aa, Komagataella pastoris
MAIPEEFDILVLGGGSSGSCIAGRLANLDHSLKVGLIEAGENNLNNPWVYLPGIYPRNMKLDSKTASFYTSNPSPHLNGRRAIVPCANVLGGGSSINFMMYTRGSASDYDDFQAEGWKTKDLLPLMKKTETYQRACNNPDIHGFEGPIKVSFGNYTYPVCQDFLRASESQGIPYVDDLEDLVTAHGAEHWLKWINRDTGRRSDSAHAFVHSTMRNHDNLYLICNTKVDKIIVEDGRAAAVRTVPSKPLNPKKPSHKIYRARKQIVLSCGTISSPLVLQRSGFGDPIKLRAAGVKPLVNLPGVGRNFQDHYCFFSPYRIKPQYESFDDFVRGDAEIQKRVFDQWYANGTGPLATNGIEAGVKIRPTPEELSQMDESFQEGYREYFEDKPDKPVMHYSIIAGFFGDHTKIPPGKYMTMFHFLEYPFSRGSIHITSPDPYAAPDFDPGFMNDERDMAPMVWAYKKSRETARRMDHFAGEVTSHHPLFPYSSEARALEMDLETSNAYGGPLNLSAGLAHGSWTQPLKKPTAKNEGHVTSNQVELHPDIEYDEEDDKAIENYIREHTETTWHCLGTCSIGPREGSKIVKWGGVLDHRSNVYGVKGLKVGDLSVCPDNVGCNTYTTALLIGEKTATLVGEDLGYTGEALDMTVPQFKLGTYEKTGLARF

SEQ ID NO: 10 - DNA, 1992 bp, Komagataella pastoris
atggctatccctgaagagtttgatatccttgttttaggtggtggatccagtggatcctgtattgccggaagattggccaacttggaccactccttgaaagttggtcttatcgaggcaggtgagaacaacctcaacaacccatgggtttaccttccaggtatttacccaagaaacatgaagttggactccaagactgcatccttctacacttctaacccttctcctcacttgaacggtagaagagctattgttccatgtgctaacgtcttgggtggtggttcttccattaacttcatgatgtacaccagaggttctgcttctgattatgacgacttccaagccgagggctggaaaaccaaggacttgcttccattgatgaaaaagaccgagacctaccaaagagcttgcaacaaccctgacattcacgggttcgaaggtccaatcaaggtttctttcggtaactacacctacccagtttgccaggacttcttgagagcttctgaatcccaaggtattccatacgttgacgacttggaagacttggttactgctcacggtgctgaacactggctgaaatggatcaacagagacactggtcgtcgttccgactccgctcatgcatttgtccactctactatgagaaaccacgacaacttgtacttgatttgtaacacaaaggttgacaagattattgtcgaagacggaagagctgctgctgttagaactgttccaagcaagcctttgaacccaaagaagccaagtcacaagatctaccgtgctagaaagcaaatcgttttgtcttgtggtaccatctcatctcctttggttctgcaaagatccggtttcggtgacccaatcaagttgagagccgctggtgttaagcctttggtcaacttgcctggtgtcggaagaaacttccaagaccactactgtttcttcagtccttacagaatcaagcctcagtacgaatctttcgatgacttcgtgcgtggtgatgctgagatccaaaagagagttttcgaccaatggtacgccaatggtactggtcctcttgccactaacggtatcgaagccggtgtcaagattagaccaacaccagaggaactgtctcaaatggacgaatctttccaagagggttacagagaatactttgaggacaagccagacaagccagttatgcactactccattattgctggtttcttcggtgaccacaccaagattcctcctggaaagtacatgaccatgttccactttttggaatacccattctccagaggttccattcacattacctctccagatccatacgcagctccagacttcgacccaggtttcatgaacgatgaaagagacatggctcctatggtctgggcctacaagaagtctagagagacagctagaagaatggaccactttgccggtgaggttacttctcaccacccattgttcccatactcatccgaggccagagctttggagatggatttggagacctccaatgcctacggtggacctttgaacttgtctgctggtcttgcccacggttcttggactcaacctttgaagaagccaactgcaaagaacgaaggccatgttacctccaaccaagtcgagcttcatccagacatcgagtacgacgaggaggacgacaaggccattgaaaactacatccgtgagcacactgagaccacatggcactgtctgggaacctgttccatcggtccaagagagggttccaagatcgtcaaatggggtggtgttttggaccacagatccaacgtttacggagtcaagggcctgaaggttggtgacttgtctgtctgtccagacaatgttggttgtaacacctacaccaccgctcttttgatcggtgagaagactgccactttggttggagaagacttaggatacaccggtgaagccttagacatgactgttcctcagttcaagttgggcacttacgagaagaccggtcttgctagattctaa

SEQ ID NO: 11 - protein, 663 aa, Komagataella pastoris
MAIPEEFDILVLGGGSSGSCIAGRLANLDHSLKVGLIEAGENNLNNPWVYLPGIYPRNMKLDSKTASFYTSNPSPHLNGRRAIVPCANILGGGSSINFMMYTRGSASDYDDFEAEGWKTKDLLPLMKKTETYQRACNNPEIHGFEGPIKVSFGNYTYPVCQDFLRATESQGIPYVDDLEDLETAHGAEHWLKWINRDTGRRSDSAHAFVHSTMRNHDNLYLICNTKVDKIIVEDGRAAGVRTVPSKPLNAKKPTHKVYRARKQIVLSCGTISSPLVLQRSGFGDPIKLRAAGVKPLVNLPGVGRNFQDHYCFFSPYRIKPQYESFDDFVRGDANIQKKVFDQWYANGTGPLATNGIEAGVKIRPTPEELSQMDESFQEGYREYFEDKPDKPVMHYSIIAGFFGDHTKIPPGKYMTMFHFLEYPFSRGSIHITSPDPYATPDFDPGFMNDERDMAPMVWSYKKSRETARKMDHFAGEVTSHHPLFPYSSEARAYEMDLETSNAYGGPLNLTAGLAHGSWTQPLKKPAARNEGHVTSNQVELHPDIEYDEEDDKAIENYIREHTETTWHCLGTCSIGPREGSKIVKWGGVLDHRSNVYGVKGLKVGDLSVCPDNVGCNTYTTALLIGEKTATLVGEDLGYTGDALDMTVPQFKLGTYEKTGLARF

SEQ ID NO: 12 - DNA, 1992 bp, Komagataella pastoris
atggctattcctgaagaattcgatattcttgtcctaggtggtggatccagtggatcctgtattgccggaagattggccaacttggaccactctttgaaagttggtcttatcgaggccggtgagaacaatcttaacaacccttgggtctaccttccaggtatttacccaagaaacatgaaattggactccaagaccgcttctttctacacctccaacccatctcctcatttgaatggtagaagagctattgtcccatgtgctaacatcttgggtggtggttcttccatcaacttcatgatgtacaccagaggttccgcttctgattacgatgacttcgaagctgagggctggaaaaccaaggatttgcttcctttgatgaagaagactgagacctaccaaagagcttgcaacaaccctgagatccacggtttcgaaggtccaatcaaggtttctttcggtaactacacttacccggtttgtcaagacttcttgagagcaactgaatcccaaggtattccatacgttgacgacttggaagacttggagactgctcatggtgccgaacactggttgaaatggatcaacagagacactggtcgtcgttccgactctgctcatgctttcgtccattctactatgagaaaccatgataacttgtacttgatctgcaacaccaaggttgacaagattattgttgaagacggaagagctgctggtgtcagaaccgtcccaagtaaacctttgaacgcaaagaagccaactcacaaggtttaccgtgctagaaagcagatcgttttgtcttgtggtaccatttcttcccctctggttttgcaaagatccggttttggtgatccaatcaaattgagagccgctggtgttaagcctttggtcaacttgccaggtgttggaaggaacttccaggaccattactgcttcttctctccttacagaatcaagccccaatacgagtcttttgatgacttcgtccgtggtgacgctaacatccaaaagaaggtattcgaccaatggtacgctaacggtactggtccattggccaccaatggtattgaagccggtgtcaagatcagaccaactccagaggaattatctcaaatggacgagtcgttccaggagggttacagagagtactttgaagacaaaccagacaaaccagttatgcactattccatcattgctggtttcttcggtgaccacaccaagattccgcctggaaagtacatgaccatgttccacttcttggagtacccattctccagaggttctattcatatcacctctccagacccatacgcaactccagactttgacccaggtttcatgaatgatgaaagagacatggctcctatggtttggtcttacaagaagtccagagagactgccagaaagatggatcactttgctggtgaggttacttcccaccaccctctgttcccatactcatccgaggccagagcttacgagatggacttggagacctccaacgcctacggtggaccactgaacttgactgctggtcttgctcacggttcttggactcagcctttgaagaagcctgccgcaagaaacgaaggacatgttacctctaaccaagttgagcttcatccagacattgaatacgatgaggaggatgacaaggccattgagaactacatccgtgagcacactgagaccacatggcactgtctcggaacctgttccatcggtccaagagaaggttccaagatagtcaaatggggtggtgttttggaccacagatccaacgtttacggagtcaagggcctgaaggttggtgacttgtctgtctgcccagacaatgttggttgtaacacctacaccaccgctcttttaatcggtgaaaagactgcaaccttggtgggtgaagacttaggatacacaggtgatgccttagacatgactgttcctcagttcaagttgggcacttacgagaagactggtcttgctagattctag

SEQ ID NO: 13 - protein, 664 aa, Ogataea methanolica
MAIPDEFDIIVVGGGSTGCALAGRLGNLDENVTVALIEGGENNINNPWVYLPGVYPRNMRLDSKTATFYSSRPSPHLNGRRAIVPCANILGGGSSINFLMYTRASASDYDDWESEGWTTDELLPLMKKIETYQRPCNNRELHGFDGPIKVSFGNYTYPNGQDFIRAAESQGIPFVDDAEDLKCSHGAEHWLKWINRDLGRRSDSAHAYIHPTMRNKQNLFLITSTKCEKIIIENGVATGVKTVPMKPTGSPKTQVARTFKARKQIIVSCGTISSPLVLQRSGIGSAHKLRQVGIKPIVDLPGVGMNFQDHYCFFTPYHVKPDTPSFDDFVRGDKAVQKSAFDQWYANKDGPLTTNGIEAGVKIRPTEEELATADDEFRAAYDDYFGNKPDKPLMHYSLISGFFGDHTKIPNGKYMCMFHFLEYPFSRGFVHVVSPNPYDAPDFDPGFMNDPRDMWPMVWSYKKSRETARRMDCFAGEVTSHHPHYPYDSPARAADMDLETTKAYAGPDHFTANLYHGSWTVPIEKPTPKNAAHVTSNQVEKHRDIEYTKEDDAAIEDYIREHTETTWHCLGTCSMAPREGSKVVPTGGVVDSRLNVYGVEKLKVADLSICPDNVGCNTYSTALLIGEKASTLVAEDLGYSGDALKMTVPNFKLGTYEEAGLARF

SEQ ID NO: 14 - DNA, 1995 bp, Ogataea methanolica
atggctattccagatgaatttgatattattgttgtcggtggtggttccaccggttgtgctcttgctggtagattaggtaacttggacgaaaacgtcacagttgctttaatcgaaggtggtgaaaacaacatcaacaacccatgggtttacttaccaggtgtttatccaagaaacatgagattagactcaaagactgctactttttactcttcaagaccatcaccacacttgaacggtagaagagctattgttccatgtgctaacatcttgggtggtggttcttccatcaacttcttgatgtacaccagagcctctgcctccgattacgatgattgggaatctgaaggttggactaccgatgaattattaccactaatgaagaagattgaaacttatcaaagaccatgtaacaacagagaattgcacggtttcgatggtccaattaaggtttcatttggtaactatacttatccaaacggtcaagatttcattagagctgccgaatctcaaggtattccatttgttgatgatgctgaagatttgaaatgttcccacggtgctgagcactggttgaagtggatcaacagagacttaggtagaagatccgattctgctcatgcttacattcacccaaccatgagaaacaagcaaaacttgttcttgattacttccaccaagtgtgaaaagattatcattgaaaacggtgttgctactggtgttaagactgttccaatgaagccaactggttctccaaagacccaagttgctagaactttcaaggctagaaagcaaattattgtttcttgtggtactatctcatcaccattagttttgcaaagatctggtatcggttccgctcacaagttgagacaagttggtattaaaccaattgttgacttaccaggtgttggtatgaacttccaagatcactactgtttcttcactccataccatgtcaagccagatactccatcattcgatgactttgttagaggtgataaagctgttcaaaaatctgctttcgaccaatggtatgctaacaaggatggtccattaaccactaatggtattgaggcaggtgttaagattagaccaactgaagaagaattagccactgctgatgacgaattcagagctgcttatgatgactactttggtaacaagccagataagccattaatgcactactctctaatttctggtttctttggtgaccacaccaagattccaaacggtaagtacatgtgcatgttccacttcttggaatatccattctccagaggtttcgttcacgttgtttctccaaacccatacgatgctcctgactttgatccaggtttcatgaacgatccaagagatatgtggccaatggtttggtcttacaagaagtccagagaaactgccagaagaatggactgttttgccggtgaagttacttctcaccacccacactacccatacgactcaccagccagagctgctgacatggacttggaaactactaaagcttatgctggtccagaccactttactgctaacttgtaccacggttcatggactgttccaattgaaaagccaactccaaagaacgctgctcacgttacttctaaccaagttgaaaaacatcgtgacatcgaatacaccaaggaggatgatgctgctatcgaagattacatcagagaacacactgaaaccacatggcattgtcttggtacttgttcaatggctccaagagaaggttctaaggttgtcccaactggtggtgttgttgactccagattaaacgtttacggtgttgaaaagttgaaggttgctgatttatcaatttgcccagataatgttggttgtaacacttactctactgctttgttaatcggtgaaaaggcttctaccttagttgctgaagacttgggctactctggtgatgctttgaagatgactgttccaaacttcaaattgggtacttatgaagaagctggtctagctagattctag

SEQ ID NO: 15 - protein, 663 aa, Ogataea methanolica
MAIPEEFDIIVVGGGSAGCPTAGRLANLDPNLTVALIEAGENNINNPWVYLPGVYPRNMRLDSKTATFYSSRPSPHLNGRRAIVPCANILGGGSSINFMMYTRGSASDYDDWESEGWTTDELLPLMKRLETYQRPCNNPDLHGFDGPIKVSFGNYTYPNCQDFLRAAESQGIPFVDDAEDLKTSHASQHWLKWINRDLGRRSDAAHAYIHPTMRNKSNLYLITSTKADKVIIEDGVAAGIQVVPSKPLNPEKPAAKIYKARKQIILSCGTISTPLVLQRSGIGSAHKLRQAGIKPIVDLPGVGMNFQDHYCFFTPYHVKPDTPSFDDFARGDKAVQKSAFDQWYANKDGPLTTNGIEAGVKIRPTAEELATADEDFQLGYASYFENKPDKPLMHYSLISGFFGDHTKIPNGKYMTMFHFLEYPFSRGFVHVVSPSPYDAPDFDPGFMNDPKDMWPMVWAYKMSRETARRMECFAGEVTSHHPKYPYDSPARAKDLDLETCKAYAGPDHFTANLYHGSWTIPLEKPTPKNTSHVTSNQVELHAQLEYSKEDDIAIENYIKEHVETTWHCLGTCSMAPREGSSIVPTGGVVDERLNVYDVAHLKCADLSICPDNVGCNTYSTALLVGEKASMIVAEDLGYSGAELDMTIPGFKLGTYESTGLGRF

SEQ ID NO: 16 - DNA, 1992 bp, Ogataea methanolica
atggctattcctgaagaattcgatatcattgttgtcggtggtggttctgccggctgtcctactgctggtagattggctaacttagacccaaatttaactgttgctttaatcgaagctggtgaaaacaacattaacaacccatgggtctacttaccaggcgtttacccaagaaacatgagattagactccaaaactgcaactttctactcttctagaccttccccacatttaaatggtagaagagctattgttccatgtgctaatatcttaggtggtggttcttcaattaacttcatgatgtacactagaggttcagcttctgattatgatgactgggaatccgaaggttggactaccgatgaattattgccattgatgaaaagattagaaacttatcaaagaccatgtaacaaccctgatttgcacggtttcgacggccctatcaaggtctccttcggtaactacacttatcctaactgtcaagatttcttaagagccgctgaatctcaaggtattccatttgttgatgatgctgaagatttaaagacttctcatgcttcccaacactggctgaagtggattaacagagacctgggtagaagatctgatgctgcgcatgcttacattcacccaactatgagaaacaagtcaaacttatacttgatcacttccactaaggctgataaagttataattgaagatggagttgcagctggtattcaagttgttccttccaaaccattgaacccagaaaagccggctgccaagatctacaaggctagaaagcaaatcattctatcctgtggtacaatttctaccccgttggtcctacaaagatctggtattggctcagctcataaattaagacaggcaggcataaaaccgatcgttgacttgccaggagttggtatgaacttccaagatcactactgctttttcaccccataccatgtcaagccagatactccttcttttgatgactttgccagaggtgataaggctgttcaaaaatcagcttttgatcaatggtatgctaacaaagatggtcctttaaccactaacggtattgaagctggtgttaagattagaccaactgctgaagaactggctactgctgatgaagatttccaactaggctacgcttcttactttgaaaacaagccagataaaccattgatgcattactctttaatctctggtttctttggtgatcacactaagattccaaacggtaaatacatgaccatgttccatttcttagaatacccattctccaggggttttgttcacgttgtttcgccaagcccatacgatgctccagactttgacccaggtttcatgaacgacccaaaggacatgtggccaatggtttgggcttataaaatgtcaagagaaactgctagaagaatggaatgctttgctggtgaagttacttcccaccatcctaaatatccatacgattcacctgccagagctaaggacttggacttggaaacttgtaaagcttacgcgggtccagatcactttactgcaaacttgtaccacggttcgtggaccattccattggagaagccaactcccaagaacacttctcacgttacttcgaatcaagttgaattacatgctcaattagaatattctaaagaagatgacatcgccatcgaaaactatatcaaggaacacgttgaaactacctggcattgtcttggtacttgttcaatggctccaagagaaggctcatcaattgtcccaacaggtggtgttgttgatgaaagactaaacgtttatgatgttgctcacttaaaatgtgctgatttatctatctgtccagataatgtgggttgtaacacttactctactgcgttactggttggtgaaaaggcttctatgattgttgctgaagatttaggttactctggagctgaattggatatgaccattcctggtttcaagttaggtacttacgaatctactggattaggtagattctaa

SEQ ID NO: 17 - DNA, 1000 bp, Ogataea methanolica
gacaaagttttgttaaatgactatcgaacaagccatgaaatagcacatttctgccagtcacttttaacactttcctgcttgctggttgactctcctcatacaaacacccaaaagggaaactttcagtgtggggacacttgacatctcacatgcaccccagattaatttccccagacgatgcggagacaagacaaaacaaccctttgtcctgctcttttctttctcacaccgcgtgggtgtgtgcgcaggcaggcaggcaggcagcgggctgcctgccatctctaatcgctgctcctcccccctggcttcaaataacagcctgctgctatctgtgaccagattgggacacccccctcccctccgaatgatccatcaccttttgtcgtactccgacaatgatccttccctgtcatcttctggcaatcagctccttcaataattaaatcaaataagcataaatagtaaaatcgcatacaaacgtcatgaaaagttttatctctatggccaacggatagtctatctgcttaattccatccactttgggaaccgttctctctttaccccagattctcaaagctaatatctgccccttgtctattgtcctttctccgtgtacaagcggagcttttgcctcccatcctcttgctttgtttcggttatttttttttcttttgaaactcttggtcaaatcaaatcaaacaaaaccaaaccttctattccatcagatcaaccttgttcaacattctataaatcgatataaatataaccttatccctcccttgttttttaccaattaatcaatcttcaaatttcaaatattttctacttgctttattactcagtattaacatttgtttaaaccaactataacttttaactggctttagaagttttatttaacatcagtttcaatttacatctttatttattaacgaaatctttacgaattaactcaatcaaaacttttacgaaaaaaaaatcttactattaatttctcaaa

SEQ ID NO: 18 - DNA, 1000 bp, Ogataea methanolica
cgaacttgcccttgtggaatttggttgttaatcaaactgttctgtatttcatgtcatactactattgatattattaatgttacttactcatctggccatttaacaggtttgaagctttaatgctcttaactaacagcaatccatcaccgtcaaccttaacccccctggtgcttgctgtctttatccttcgtatctttttcatgttgcaccgccctgttccttatacggttgttcccccataggctaacttctctgtttccgaccatctctgcaataacaaagaattctatacgcttacactataatcatacaatgactctacatgccattttcactttacttacttgccatcggaagatactgaatcagaaagccatagtaactacataacttcaaaacacaccctttttacagattagttacaattttgtcaatgtttgtttgataacccaaggtggaacgtttccagttagacctgtttaatccaactcactttaccaccccaaaactttcctaccgttagacaaatactggctaaatctgacgaaaacaaccaatcaacaattgaatccactgggaggtatctctaatccactgacaaactttgctaaaacaagaaaaagtgggggcctccgttgcggagaagacgtgcgcaggcttaaaaacacaagagaacacttggaagtaccccagatttttagcttcctactattctgacaccccctattcaagcacgacggtgattgattcattcaattttgctgctccaatgataggataaacccttttggacttcaatcagacctctgtcctccatagcaatataaataccttctagttgccccacttcctctctcctgtactgccccaatgagtgacttattcaagttactttctctcttttcctaacaattaaacaagaagctttattataacattaatatactattttataacaggattgaaaattatatttatctatctaaaactaaaattcaaa

SEQ ID NO: 19 - protein, 664 aa, Ogataea polymorpha
MAIPDEFDIIVVGGGSTGCCIAGRLANLDDQNLTVALIEGGENNINNPWVYLPGVYPRNMRLDSKTATFYSSRPSKALNGRRAIVPCANILGGGSSINFLMYTRASASDYDDWESEGWSTDELLPLIKKIETYQRPCNNRDLHGFDGPIKVSFGNYTYPTCQDFLRAAESQGIPVVDDLEDFKTSHGAEHWLKWINRDLGRRSDSAHAYVHPTMRNKQSLFLITSTKCDKVIIEDGKAVAVRTVPMKPLNPKKPVSRTFRARKQIVISCGTISSPLVLQRSGIGAAHHLRSVGVKPIVDLPGVGENFQDHYCFFTPYYVKPDVPTFDDFVRGDPVAQKAAFDQWYSNKDGPLTTNGIEAGVKIRPTEEELATADEDFRRGYAEYFENKPDKPLMHYSVISGFFGDHTKIPNGKFMTMFHFLEYPFSRGFVRITSANPYDAPDFDPGFLNDERDLWPMVWAYKKSRETARRMESFAGEVTSHHPLFKVDSPARARDLDLETCSAYAGPKHLTANLYHGSWTVPIDKPTPKNDFHVTSNQVQLHSDIEYTEEDDEAIVNYIKEHTETTWHCLGTCSMAPREGSKIAPKGGVLDARLNVYGVQNLKVADLSVCPDNVGCNTYSTALTIGEKAATLVAEDLGYSGSDLDMTIPNFRLGTYEETGLARF

SEQ ID NO: 20 - DNA, 1995 bp, Ogataea polymorpha
atggccattcctgacgaattcgatatcattgttgttggtggaggttccaccggctgctgcattgcgggcagactcgcaaacctcgacgaccaaaacctcacagttgccctgatcgagggtggtgagaacaacatcaacaacccttgggtctaccttcccggagtgtatcctagaaacatgagactcgactccaagacggccaccttctactcgtccagaccatcgaaggctctgaacggcagaagagcgatcgttccttgcgccaacatccttggaggcggctcgtcgatcaactttctgatgtacaccagagcctctgcttccgactacgacgactgggagtccgagggatggagcaccgacgagttgctacctctgatcaaaaaaatcgaaacttaccagcgtccttgcaacaacagagatctgcacggctttgacggcccaatcaaggtttcctttggaaactacacgtatcctacgtgccaggacttcctgagagcagcagagtcgcagggaattcctgttgtggacgacctggaggacttcaagacatcgcatggtgcagagcactggctgaagtggattaacagagacctgggcagaagatcggattctgcgcacgcctacgtccacccaactatgagaaacaagcagagcctgttcctcatcacctccaccaagtgtgacaaggtgatcatcgaggacggcaaggctgtggccgtgagaacagtgccaatgaagcctctgaaccctaagaagcctgtgtccagaaccttcagagccagaaagcagattgtgatctcctgcggaaccatctcgtctcctctggtgctccagagatctggtattggtgcagctcaccacttgagatccgtgggggtcaagccaatcgtcgacctgccaggtgtgggtgagaatttccaggaccactactgtttcttcactccatactacgtcaagcctgacgttcctacgttcgacgactttgtcaggggtgacccagttgcccagaaggccgctttcgaccagtggtactccaacaaggacggtccattgaccaccaacggtattgaagccggagtcaagatcagacctaccgaagaggagctggctaccgcggacgaggacttcagacgcggctacgcagagtacttcgagaacaagccagacaagcctctgatgcactactctgtcatctccggcttctttggagaccacaccaagattcctaacggcaagttcatgaccatgttccacttcctggagtatccattctccagaggatttgttagaatcacctcggcaaacccatacgacgctcctgacttcgatcccggcttcctcaatgacgaaagagacctgtggcctatggtctgggcatacaagaagtccagagagacggccagaagaatggagagctttgcaggagaggtcacctcgcaccacccattgttcaaggttgactcgccagccagagccagagacctggacctcgagacatgcagtgcatatgccggtcctaagcacctcactgccaacctgtaccacggctcgtggaccgttcctatcgacaagccaacgcctaagaacgatttccacgtgacctccaaccaagtccaactgcactccgacatcgagtacaccgaggaggacgacgaggccatcgtcaactacattaaggaacacaccgagaccacttggcactgtctgggtacctgctcgatggccccaagagagggtagtaagattgctcctaagggaggtgtcttggacgccagactgaacgtttacggagtccagaacctcaaggttgcggacctttctgtttgtcccgacaacgttggatgcaacacctactctactgcattgaccatcggtgagaaggctgccactcttgttgctgaagatcttggctactcaggctccgacctggacatgacgattccaaacttcagactcggaacttacgaggagaccggacttgccagattctaa

SEQ ID NO: 21 - DNA, 1000 bp, Ogataea polymorpha
gctgcagcttgcgatctcggatggttttggaatggaagaaccgcgacatctccaacagctgggccgtgttgagaatgagccggacgtcgttgaacgagggggccacaagccggcgtttgctgatggcgcggcgctcgtcctcgatgtagaaggccttttccagaggcagtctcgtgaagaagttgccaacgctcggaaccagctgcacgagccgagacaattcgggggtgccggctttggtcatttcaatgttgtcgtcgatgaggagttcaaggtcgtggaagatttccgcgtagcggcgttttgcctcagagtttaccatgaggtcgtccactgcagagatgccgttgctcttcaccgcgtacaggacgaacggcgtggccagcaggcccttgatccattctatgaggccatctcgacggtgttccttgagtgcgtactccactctgtagcgactggacatctcgagactgggcttgctgtgctggatgcaccaattaattgttgccgcatgcatccttgcaccgcaagtttttaaaacccactcgctttagccgtcgcgtaaaacttgtgaatctggcaactgagggggttctgcagccgcaaccgaacttttcgcttcgaggacgcagctggatggtgtcatgtgaggctctgtttgctggcgtagcctacaacgtgaccttgcctaaccggacggcgctacccactgctgtctgtgcctgctaccagaaaatcaccagagcagcagagggccgatgtggcaactggtggggtgtcggacaggctgtttctccacagtgcaaatgcgggtgaaccggccagaaagtaaattcttatgctaccgtgcagtgactccgacatccccagtttttgccctacttgatcacagatggggtcagcgctgccgctaagtgtacccaaccgtccccacacggtccatctataaatactgctgccagtgcacggtggtgacatcaatctaaagtacaaaaacaaa

SEQ ID NO: 22 - protein, 20 aa, Artificial Sequence
  Signal sequence
  MISC_FEATURE (3)..(3): X at position 3 is either F or L
  MISC_FEATURE (16)..(16): X at position 16 is either A or T
MKXSTNLILAIAAASXVVSA

SEQ ID NO: 23 - protein, 36 aa, Artificial Sequence
  Leader sequence
  MISC_FEATURE (3)..(3): X at position 3 is either F or L
  MISC_FEATURE (16)..(16): X at position 16 is either A or T
MKXSTNLILAIAAASXVVSAAPVAPAEEAANHLHKR

SEQ ID NO: 24 - protein, 85 aa, Saccharomyces cerevisiae
MRFPSIFTAVLFAASSALAAPVNTTTEDETAQIPAEAVIGYSDLEGDFDVAVLPFSNSTNNGLLFINTTIASIAAKEEGVSLEKR

SEQ ID NO: 25 - DNA, 1991 bp, Artificial Sequence
  AOX1 split marker cassette 1
aggggtccaagtaagaagcttcttgctgtagaatttgggcatatgtgctggtgacaaaggcatctctgccttgagtttctgacggcgggacagcattcttaccggatatataacaccaattgccagcaccaccaatctcagaggtacccctaacaaacttaataaaatcttgggtatcaacttcattaagctttgtagtttgcaagtacttataaacaaaattccgtaaggtgtcgtcttgaggctgggacttgacaaactgccaaaatggcaacaaatctactggcttggccataattttgacattcgagtcatcaaaggtaaattcaaccggagacttgtattctttattgataactttctcatataggacattgtcaggaacacgatgaaaccaggatgcccccaaatccaatgagactgaggtttcatgagtcgcaaccaacctacctccaatacggtccctaccctctaaaatcaacgcattcacgccattgcttttgagatcgactgcagctttgatgcctgaaatcccagcgcctacaatgatgacatttggatttggttgactcatgttggtattgtgaaatagacgcagatcgggaacactgaaaaataacagttattattcgagatctaacatccaaagacgaaaggttgaatgaaacctttttgccatccgacatccacaggtccattctcacacataagtgccaaacgcaacaggaggggatacactagcagcagaccgttgcaaacgcaggacctccactcctcttctcctcaacacccacttttgccatcgaaaaaccagcccagttattgggcttgattggagctcgctcattccaattccttctattaggctactaacaccatgactttattagcctgtctatcctggcccccctggcgaggttcatgtttgtttatttccgaatgcaacaagctccgcattacacccgaacatcactccagatgagggctttctgagtgtggggtcagtacgctgcaggtcgacaacccttaatataacttcgtataatgtatgctatacgaagttattaggtctagatcggtaccgacatggaggcccagaataccctccttgacagtcttgacgtgcgcagctcaggggcatgatgtgactgtcgcccgtacatttagcccatacatccccatgtataatcatttgcatccatacattttgatggccgcacggcgcgaagcaaaaattacggctcctcgctgcagacctgcgagcagggaaacgctcccctcacagacgcgttgaattgtccccacgccgcgcccctgtagagaaatataaaaggttaggatttgccactgaggttcttctttcatatacttccttttaaaatcttgctaggatacagttctcacatcacatccgaacataaacaaccatgggtaaggaaaagactcacgtttcgaggccgcgattaaattccaacatggatgctgatttatatgggtataaatgggctcgcgataatgtcgggcaatcaggtgcgacaatctatcgattgtatgggaagcccgatgcgccagagttgtttctgaaacatggcaaaggtagcgttgccaatgatgttacagatgagatggtcagactaaactggctgacggaatttatgcctcttccgaccatcaagcattttatccgtactcctgatgatgcatggttactcaccactgcgatccccggcaaaacagcattccaggtattagaagaatatcctgattcaggtgaaaatattgttgatgcgctggcagtgttcctgcgccggttgcattcgattcctgtttgtaattgtccttttaacagcgatcgcgtatttcgtctcgctcaggcgcaatcacgaatgaataacggtttggttgatgcgagtgattttgatgacgagcgtaatggctggcctgttgaacaagtctggaaagaaatgcataagcttttgccattctcaccg

SEQ ID NO: 26 - DNA, 1853 bp, Artificial Sequence
  AOX1 split marker cassette 2
aagcccgatgcgccagagttgtttctgaaacatggcaaaggtagcgttgccaatgatgttacagatgagatggtcagactaaactggctgacggaatttatgcctcttccgaccatcaagcattttatccgtactcctgatgatgcatggttactcaccactgcgatccccggcaaaacagcattccaggtattagaagaatatcctgattcaggtgaaaatattgttgatgcgctggcagtgttcctgcgccggttgcattcgattcctgtttgtaattgtccttttaacagcgatcgcgtatttcgtctcgctcaggcgcaatcacgaatgaataacggtttggttgatgcgagtgattttgatgacgagcgtaatggctggcctgttgaacaagtctggaaagaaatgcataagcttttgccattctcaccggattcagtcgtcactcatggtgatttctcacttgataaccttatttttgacgaggggaaattaataggttgtattgatgttggacgagtcggaatcgcagaccgataccaggatcttgccatcctatggaactgcctcggtgagttttctccttcattacagaaacggctttttcaaaaatatggtattgataatcctgatatgaataaattgcagtttcatttgatgctcgatgagtttttctaatcagtactgacaataaaaagattcttgttttcaagaacttgtcatttgtatagtttttttatattgtagttgttctattttaatcaaatgttagcgtgatttatattttttttcgcctcgacatcatctgcccagatgcgaagttaagtgcgcagaaagtaatatcatgcgtcaatcgtatgtgaatgctggtcgctatactggtaccattcgagaacccttaatataacttcgtataatgtatgctatacgaagttattaggtgatatcagatccactgccatttgcctgagagatgcaggcttcatttttgatacttttttatttgtaacctatatagtataggattttttttgtcattttgtttcttctcgtacgagcttgctcctgatcagcctatctcgcagctgatgaatatcttgtggtaggggtttgggaaaatcattcgagtttgatgtttttcttggtatttcccactcctcttcagagtacagaagattaagtgagacgttcgtttgtgcaagcttcaacgatgccaaaagggtataataagcgtcatttgcagcattgtgaagaaaactatgtggcaagccaagcctgcgaagaatgtattttaagtttgactttgatgtattcacttgattaagccataattctcgagtatctatgattggaagtatgggaatggtgatacccgcattcttcagtgtcttgaggtctcctatcagattatgcccaactaaagcaaccggaggaggagatttcatggtaaatttctctgacttttggtcatcagtagactcgaactgtgagactatctcggttatgacagcagaaatgtccttcttggagacagtaaatgaagtcccaccaataaagaaatccttgttatcaggaacaaacttcttgtttcgaactttttcggtgccttgaactataaaatgtagagtggatatgtcgggtaggaatggagcgggcaaatgcttaccttctggaccttcaagaggtatgtagggtttgtagatactgatgccaacttcagtgacaacgttgctatttcgttcaaaccattccgaatccagagaaatcaaagttgtttgtctactattgatccaagccagtgcggtcttgaaactgacaatagtgtgctcgtgttttgaggtcatctttgt

SEQ ID NO: 27 - DNA, 2038 bp, Artificial Sequence
  AOX2 split marker cassette 1
gtacgggtttactgatttgacatatcttggtactaacgttaccaatggtgttccaaataacgcagatgatgagcgtggttgcattgctggatttgacaacactggtttcgtgctgggaacttcatcctcgttgtttaatcagtttattctgcaactgaatacgagtgatctttcaggagcaatttaccaaatcattgagcattttctgactggacttagcgaagacgaagacgacattgctatctattcccccaaccctttctacaaaagtacgtatgcaggagtaggtgccattgcggaaaatgacaccctttacttggttgatggtggagaggataaccaaaacgtccctctgcagcctctacttcaaaaggagcgtgacgttgatatcatctttgcgtttgacaacagtgcagacactgacctctcttggccaaacggttcatcattagtcaacacctacatgagacagttttcttctcaagcaaatggaacaacgttcccttatgtacctgataccaccactttcctaaacttgaatctttcgagtaagccaaccttctttggttgtgatgctagaaatttgacagacattgttgaaggcacggatcacattcctcccctggttgtttatctggccaatagacctttctcgtattggagtaacacttcaactttcaagttagactactctgaatccgagaagagaggaatgatccaaaacggttttgaagtgtcgtctcgtttgaacatgactattgatgaagaatggcgtacttgtgttggatgtgcaatcattcgtagacagcaggagagatccaatgcaacacaaacagagcaatgtagaagatgttttgagaattattgttggaacggtgatattgacacttccaccgaagatatccccgttaattttaccactactggagcaaccaatgaggagaatgacaactccacttcaatatcatcggccaattcggtagcaccttccaaactttggtaccaagcaccattgctgttggtcggccttgtcgcattcttcatctagtacgtacgctgcaggtcgacaacccttaatataacttcgtataatgtatgctatacgaagttattaggtctagatcggtaccgacatggaggcccagaataccctccttgacagtcttgacgtgcgcagctcaggggcatgatgtgactgtcgcccgtacatttagcccatacatccccatgtataatcatttgcatccatacattttgatggccgcacggcgcgaagcaaaaattacggctcctcgctgcagacctgcgagcagggaaacgctcccctcacagacgcgttgaattgtccccacgccgcgcccctgtagagaaatataaaaggttaggatttgccactgaggttcttctttcatatacttccttttaaaatcttgctaggatacagttctcacatcacatccgaacataaacaaccatgggtaaggaaaagactcacgtttcgaggccgcgattaaattccaacatggatgctgatttatatgggtataaatgggctcgcgataatgtcgggcaatcaggtgcgacaatctatcgattgtatgggaagcccgatgcgccagagttgtttctgaaacatggcaaaggtagcgttgccaatgatgttacagatgagatggtcagactaaactggctgacggaatttatgcctcttccgaccatcaagcattttatccgtactcctgatgatgcatggttactcaccactgcgatccccggcaaaacagcattccaggtattagaagaatatcctgattcaggtgaaaatattgttgatgcgctggcagtgttcctgcgccggttgcattcgattcctgtttgtaattgtccttttaacagcgatcgcgtatttcgtctcgctcaggcgcaatcacgaatgaataacggtttggttgatgcgagtgattttgatgacgagcgtaatggctggcctgttgaacaagtctggaaagaaatgcataagcttttgccattctcaccg

SEQ ID NO: 28 - DNA, 1944 bp, Artificial Sequence
  AOX2 split marker cassette 2
aagcccgatgcgccagagttgtttctgaaacatggcaaaggtagcgttgccaatgatgttacagatgagatggtcagactaaactggctgacggaatttatgcctcttccgaccatcaagcattttatccgtactcctgatgatgcatggttactcaccactgcgatccccggcaaaacagcattccaggtattagaagaatatcctgattcaggtgaaaatattgttgatgcgctggcagtgttcctgcgccggttgcattcgattcctgtttgtaattgtccttttaacagcgatcgcgtatttcgtctcgctcaggcgcaatcacgaatgaataacggtttggttgatgcgagtgattttgatgacgagcgtaatggctggcctgttgaacaagtctggaaagaaatgcataagcttttgccattctcaccggattcagtcgtcactcatggtgatttctcacttgataaccttatttttgacgaggggaaattaataggttgtattgatgttggacgagtcggaatcgcagaccgataccaggatcttgccatcctatggaactgcctcggtgagttttctccttcattacagaaacggctttttcaaaaatatggtattgataatcctgatatgaataaattgcagtttcatttgatgctcgatgagtttttctaatcagtactgacaataaaaagattcttgttttcaagaacttgtcatttgtatagtttttttatattgtagttgttctattttaatcaaatgttagcgtgatttatattttttttcgcctcgacatcatctgcccagatgcgaagttaagtgcgcagaaagtaatatcatgcgtcaatcgtatgtgaatgctggtcgctatactggtaccattcgagaacccttaatataacttcgtataatgtatgctatacgaagttattaggtgatatcagatccacttcctcttacggctttctttcccaaaaaatcattggggaaatgtgcccctcatcagagtccaatgacccatgaataaagtttcttgtactgtttaagacgatgaattgcaacgataatccgagcagtttacggggtacatcacgtgctttgcatatgatctcggagtcggatcagttccggatgtgatgtattaccccatagtttcaaactctaatgcagccgccaagtgccatacaccctccatcaatctatgcttaaagtttttcaccatcgttgggtggtgatgatgactcgcttagtctctgctgttcgatattaactttgtaaggatcgcccttggatggaaaattgaggggttgtaacctgaatttgcaggctacttacattggacttttgagaaggctggacggttgatgaagagggctgggtgcagaggaatggaaaaaaatttagttgagaggactgcttgaaattttaggaaatggagtcctttaagctgacaaaacttcaaggatggggattttcatgtagctttttcatgccttcgacaagctaaaggaaggtaattgattctggataaatggatatttgatctgctttagcagatgtcaaagttctactagtgatagtctggtatctcgtagccttcaattgggcgtatcttactcgaagtgttatatttttagctgacgagacgaagaacgagagagtattgacacattcagaggtaagacaatatgtcgtattatcaaaataagtatcgaacctctattaggagcctactggctcaaatgtgcaaccttagtggtgattgtctctgcttcttgatcacaatctgtcgtgtttgagagtgccgatgtatgatttttagtaaatgtttttcagaaaaggcgctaagtaaataaccagtaagtaataaataacgtaaaagtgatttgaatcataaaagaatcaagatagaggtcaaagcatagataatccccc

SEQ ID NO: 29 - DNA, 22 bp, Artificial Sequence
  Primer sequence
ggctggaaatagatgtagggag

SEQ ID NO: 30 - DNA, 21 bp, Artificial Sequence
  Primer sequence
tcgcatctccgcaaatttctc

SEQ ID NO: 31 - DNA, 21 bp, Artificial Sequence
  Primer sequence
gatcccattccctatccatgt

SEQ ID NO: 32 - DNA, 20 bp, Artificial Sequence
  Primer sequence
ctctcccccctcgtaatctt

SEQ ID NO: 33 - DNA, 720 bp, Artificial Sequence
  enhanced green fluorescent protein (eGFP)
atggtgagcaagggcgaggagctgttcaccggggtggtgcccatcctggtcgagctggacggcgacgtaaacggccacaagttcagcgtgtccggcgagggcgagggcgatgccacctacggcaagctgaccctgaagttcatctgcaccaccggcaagctgcccgtgccctggcccaccctcgtgaccaccctgacctacggcgtgcagtgcttcagccgctaccccgaccacatgaagcagcacgacttcttcaagtccgccatgcccgaaggctacgtccaggagcgcaccatcttcttcaaggacgacggcaactacaagacccgcgccgaggtgaagttcgagggcgacaccctggtgaaccgcatcgagctgaagggcatcgacttcaaggaggacggcaacatcctggggcacaagctggagtacaactacaacagccacaacgtctatatcatggccgacaagcagaagaacggcatcaaggtgaacttcaagatccgccacaacatcgaggacggcagcgtgcagctcgccgaccactaccagcagaacacccccatcggcgacggccccgtgctgctgcccgacaaccactacctgagcacccagtccgccctgagcaaagaccccaacgagaagcgcgatcacatggtcctgctggagttcgtgaccgccgccgggatcactctcggcatggacgagctgtacaagtaa

SEQ ID NO: 34 - DNA, 1830 bp, Artificial Sequence
  Human serum albumin (HSA) with its native secretion leader
atgaagtgggttactttcatctccttgttgttcttgttctcctcagcttactccagaggtgttttcagaagagatgctcacaagtccgaggttgctcacagattcaaggacttgggtgaagagaacttcaaggctttggttttgatcgctttcgctcagtacttgcagcagtgtccattcgaggaccacgttaagttggttaacgaggttactgagttcgctaagacttgtgttgctgacgaatccgctgagaactgtgataagtccttgcacactttgttcggtgacaagttgtgtactgttgctactttgagagaaacttacggtgagatggctgactgttgtgctaagcaagagcctgagagaaacgagtgtttcttgcaacacaaggacgacaacccaaacttgccaagattggttagaccagaggttgacgttatgtgtactgctttccacgacaacgaagagactttcttgaagaagtacttgtacgagatcgctagaagacacccatacttctacgctccagagttgttgttcttcgctaagagatacaaggctgctttcactgagtgttgtcaggctgctgataaggctgcttgtttgttgccaaagttggacgagttgagagatgagggtaaggcttcttccgctaagcagagattgaagtgtgcttccttgcagaagttcggagagagagcttttaaggcttgggctgttgctagattgtcccagagattcccaaaggctgagttcgctgaggtttccaagttggttactgacttgactaaggttcacacagagtgttgtcacggtgacttgttggaatgtgctgatgacagagctgacttggctaagtacatctgtgagaaccaggattccatctcctccaagttgaaagaatgttgtgagaagcctttgttggagaagtcccactgtatcgctgaggttgaaaacgacgaaatgccagctgacttgccatctttggctgctgacttcgttgaatccaaggacgtctgcaagaactacgctgaggctaaggacgttttcttgggtatgttcttgtatgagtacgctagaagacatccagactactccgttgttttgttgttgagattggctaagacttacgagactactttggagaagtgttgtgctgctgctgacccacatgagtgttacgctaaggttttcgacgagttcaagccattggttgaggaaccacagaacttgatcaagcagaactgtgagttgttcgagcagttgggtgagtacaagttccagaacgctttgttggttagatacactaagaaggttccacaggtttccactccaactttggttgaggtttccagaaacttgggtaaggttggttccaagtgttgtaagcacccagaggctaagagaatgccatgtgctgaggactacttgtctgttgttttgaaccagttgtgtgtcttgcacgaaaagacaccagtttccgacagagttactaagtgttgtactgaatccttggttaacagaagaccttgtttctccgctttggaggttgacgagacttacgttccaaaagagttcaacgctgagactttcactttccacgctgacatctgtactttgtccgagaaagagagacagatcaagaagcagactgctttggttgagttggttaagcacaagccaaaggctacaaaagagcagttgaaggctgttatggacgacttcgctgctttcgttgagaaatgttgtaaggctgacgacaaagagacttgtttcgctgaagagggtaagaagttggttgctgcttcccaagctgctttgggtctgtaa

SEQ ID NO: 35 - DNA, 1056 bp, Artificial Sequence
  variable region of a camelid antibody (VHH) with the S. cerevisiae alpha-mating factor leader
atgagattcccatctattttcaccgctgtcttgttcgctgcctcctctgcattggctgcccctgttaacactaccactgaagacgagactgctcaaattccagctgaagcagttatcggttactctgaccttgagggtgatttcgacgtcgctgttttgcctttctctaactccactaacaacggtttgttgttcattaacaccactatcgcttccattgctgctaaggaagagggtgtctctctcgagaagagacaagccggtggttcattaagattgtcctgtgctgcctctggtagaactttcacttctttcgcaatgggttggtttagacaagcacctggaaaagagagagagtttgttgcttctatctccagatccggtactttaactagatacgctgactctgccaagggtagattcactatttctgttgacaacgccaagaacactgtttctttgcaaatggacaaccttaacccagatgacaccgcagtctattactgtgccgctgacttgcacagaccatacggtccaggaacccaaagatccgatgagtacgattcttggggtcagggaactcaagtcactgtctcttcaggtggtggatctggtggtggaggttcaggtggtggaggatccggtggtggtggttctggtggtggtggatctggtggaggtgaagttcaacttgtcgaatccggtggtgcacttgtccaacctggtggatctcttagactttcttgtgccgcctccggttttcctgttaaccgttactctatgcgttggtacagacaagcccctggaaaagaacgtgaatgggttgccggaatgtcctcagctggtgacagatcctcctacgaagattctgtgaagggacgtttcaccatctccagagatgacgcccgtaacaccgtttaccttcaaatgaactcccttaagcctgaggatactgccgtctactattgtaacgtgaatgtcggatttgaatactggggacagggaacccaagttactgtctcttccggtggacatcaccaccaccatcactaatag

SEQ ID NO: 36 - DNA, 991 bp, Pichia pastoris
gcaaggcaactgagaaattgaatagtggtttcaagcccgctgactttttgtattatctcaatgtcggtgtttcacagtccccagaagggggctttgccttcaagggagacggaagagacatcgtcaaccctggggagaagtatttcaaatggcgcaagttcgctaatttttacgattaagcagtgctgtatggggtagttaataaatcgggaatatccttctgacgtgactgtaacaaatctctttttacgtggtgcgcatactggacagaggcagagtctcaatttcttcttttgagacaggctactacagcctgtgattcctcttggtacttggatttgcttttatctggctccgttgggaactgtgcctgggttttgaagtatcttgtggatgtgtttctaacactttttcaatcttcttggagtgagaatgcaggactttgaacatcgtctagctcgttggtaggtgaaccgttttaccttgcatgtggttaggagttttctggagtaaccaagaccgtcttatcatcgccgtaaaatcgctcttactgtcgctaataatcccgctggaagagaagttcgaacagaagtagcacgcaaagctcttgtcaaatgagaattgttaatcgtttgacaggtcacactcgtgggctatgtacgatcaacttgccggctgttgctggagagatgacaccagttgtggcatggccaattggtattcagccgtaccactgtatggaaaatgagattatcttgttcttgatctagtttcttgccattttagagttgccacattcgtaggtttcagtaccaataatggtaacttccaaacttccaacgcagataccagagatctgccgatccttccccaacaataggagcttactacgccatacatatagcctatctattttcactttcgcgtgggtgcttctatataaacggttccccatcttccgtttcatactacttgaattttaagcactaaa

SEQ ID NO: 37 - DNA, 864 bp, Pichia pastoris
cttttctttgggcaaggaaaaatcaagaaaaagcagaggttaaagttttcaggggaatggcaattgctttatatatgggagaaagttaactacgtcggtgctgtaggcgtagagagcgactggagaatgcgtgatgaggtcgtctcttttcgcccccccttggcggggtaaaaattgcactactgcagaattactacacccctattccgaggagacggagtgcgacaaaaatggtaaagttcaccctagtctgcgacttttaattgacggacaccggcgtttacatgcgaaaaaaactaaagtgcgcgcatttcacggccgaggggggtcccacttgggactgagagggggtgggatctgaaatcgaggaggtatcaagaccccccgtttctcaactccctaatcaaaaattacgaagtcctcgttggaaaggagttaaaataattaagcggggtcggacgccataccgaggttatcttgcaggcattttactaatattggaattcggagctcaacttgcaaccaggcagggtttagctatgtaatcaatgtaatcaatataataaagcactaccacatcgaaggtttgggagggaggccaatagtgtcccccacagggtgctgatatcgcgattcttgggtgaggagacacatatttcactcctctcaccaaccaaccaagcggctcctcgcaagatgatttatccgattatccggacactatactcccatccagtttgatgccgatttcatcgattgtcctaaataatccttaaatatgtatagaacggtaccctggggttacataatccttatttaataatccctcccccaccgcttttctttttttttcttcttattgtc

SEQ ID NO: 38 - DNA, 1000 bp, Pichia pastoris
aaatggcagaaggatcagcctggacgaagcaaccagttccaactgctaagtaaagaagatgctagacgaaggagacttcagaggtgaaaagtttgcaagaagagagctgcgggaaataaattttcaatttaaggacttgagtgcgtccatattcgtgtacgtgtccaactgttttccattacctaagaaaaacataaagattaaaaagataaacccaatcgggaaactttagcgtgccgtttcggattccgaaaaacttttggagcgccagatgactatggaaagaggagtgtaccaaaatggcaagtcgggggctactcaccggatagccaatacattctctaggaaccagggatgaatccaggtttttgttgtcacggtaggtcaagcattcacttcttaggaatatctcgttgaaagctacttgaaatcccattgggtgcggaaccagcttctaattaaatagttcgatgatgttctctaagtgggactctacggctcaaacttctacacagcatcatcttagtagtcccttcccaaaacaccattctaggtttcggaacgtaacgaaacaatgttcctctcttcacattgggccgttactctagccttccgaagaaccaataaaagggaccggctgaaacgggtgtggaaactcctgtccagtttatggcaaaggctacagaaatcccaatcttgtcgggatgttgctcctcccaaacgccatattgtactgcagttggtgcgcattttagggaaaatttaccccagatgtcctgattttcgagggctacccccaactccctgtgcttatacttagtctaattctattcagtgtgctgacctacacgtaatgatgtcgtaacccagttaaatggccgaaaaactatttaagtaagtttatttctcctccagatgagactctccttcttttctccgctagttatcaaactataaacctattttacctcaaatacctccaacatcacccacttaaaca

SEQ ID NO: 39 - DNA, 549 bp, Pichia pastoris
aatgatataaacaacaattgagtgacaggtctactttgttctcaaaaggccataaccatctgtttgcatctcttatcaccacaccatcctcctcatctggccttcaattgtggggaacaactagcatcccaacaccagactaactccacccagatgaaaccagttgtcgcttaccagtcaatgaatgttgagctaacgttccttgaaactcgaatgatcccagccttgctgcgtatcatccctccgctattccgccgcttgctccaaccatgtttccgcctttttcgaacaagttcaaatacctatctttggcaggacttttcctcctgccttttttagcctcaggtctcggttagcctctaggcaaattctggtcttcatacctatatcaacttttcatcagatagcctttgggttcaaaaaagaactaaagcaggatgcctgatatataaatcccagatgatctgcttttgaaactattttcagtatcttgattcgtttacttacaaacaactattgttgattttatctggagaataatcgaacaaa

SEQ ID NO: 40 - DNA, 1000 bp, Pichia pastoris
attactgttttgggcaatcctgttgataagacgcattctagagttgtttcatgaaagggttacgggtgttgattggtttgagatatgccagaggacagatcaatctgtggtttgctaaactggaagtctggtaaggactctagcaagtccgttactcaaaaagtcataccaagtaagattacgtaacacctgggcatgactttctaagttagcaagtcaccaagagggtcctatttaacgtttggcggtatctgaaacacaagacttgcctatcccatagtacatcatattacctgtcaagctatgctaccccacagaaataccccaaaagttgaagtgaaaaaatgaaaattactggtaacttcaccccataacaaacttaataatttctgtagccaatgaaagtaaaccccattcaatgttccgagatttagtatacttgcccctataagaaacgaaggatttcagcttccttaccccatgaacagaaatcttccatttaccccccactggagagatccgcccaaacgaacagataatagaaaaaagaaattcggacaaatagaacactttctcagccaattaaagtcattccatgcactccctttagctgccgttccatccctttgttgagcaacaccatcgttagccagtacgaaagaggaaacttaaccgataccttggagaaatctaaggcgcgaatgagtttagcctagatatccttagtgaagggttgttccgatacttctccacattcagtcatagatgggcagctttgttatcatgaagagacggaaacgggcattaagggttaaccgccaaattatataaagacaacatgtccccagtttaaagtttttctttcctattcttgtatcctgagtgaccgttgtgtttaatataacaagttcgttttaacttaagaccaaaaccagttacaacaaattataacccctctaaacactaaagttcactcttatcaaactatcaaacatcaaaa

SEQ ID NO: 41 - DNA, 1000 bp, Pichia pastoris
gtcaactgcgtactcttttgtcgaatggactactgaatctgcctcgatagccactataggaaggtccatagaggccagtttttcaactagtcttggtggaaagaaaccgacaaagcctttcatggagtcaccgatactgaaaggttcaaacaaagaatgcttgggtagtctcttaatacccatggcaacgaaaaaggggtcttcattgttcaacatgaattcgtatccacctttaatgtagtcataaagctgctgaagttccgaatcagtgatggaactgtctacagtgacaatataggagttctcaatcaccttatatccagtcgaatatatctggatagggtcgggtctcactgtggaagattcaaatgggttagatccctgtaatttcagcgatggagactcagtatgatggggcaaggaaaacggcaattggatattcaattggtcaagagatggtatcaaaagcgagtgtgccagggtagccacggtagccactgatgctaatctgataattttcatttctggagtgtcaaaacagtagtgataaaaggctatgaaggaggttgtctaggggctcgcggaggaaagtgattcaaacagacctgccaaaaagagaaaaaagagggaatccctgttctttccaatggaaatgacgtaactttaacttgaaaaataccccaaccagaagggttcaaactcaacaaggattgcgtaattcctacaagtagcttagagctgggggagagacaactgaaggcagcttaacgataacgcggggggattggtgcacgactcgaaaggaggtatcttagtcttgtaacctcttttttccagaggctattcaagattcataggcgatatcgatgtggagaagggtgaacaatataaaaggctggagagatgtcaatgaagcagctggatagatttcaaattttctagatttcagagtaatcgcacaaaacgaaggaatcccaccaagcaaaaaaaaaaatctaag

SEQ ID NO: 42 - DNA, 704 bp, Pichia pastoris
aaattaatccataagataaggcaaatgtgcttaagtaattgaaaacagtgttgtgattatataagcatggtatttgaatagaactactggggttaacttatctagtaggatggaagttgagggagatcaagatgcttaaagaaaaggattggccaatatgaaagccataattagcaatacttatttaatcagataattgtggggcattgtgacttgacttttaccaggacttcaaacctcaaccatttaaacagttatagaagacgtaccgtcacttttgcttttaatgtgatctaaatgtgatcacatgaactcaaactaaaatgatatcttttactggacaaaaatgttatcctgcaaacagaaagctttcttctattctaagaagaacatttacattggtgggaaacctgaaaacagaaaataaatactccccagtgaccctatgagcaggatttttgcatccctattgtaggcctttcaaactcacacctaatatttcccgccactcacactatcaatgatcacttcccagttctcttcttcccctattcgtaccatgcaacccttacacgccttttccatttcggttcggatgcgacttccagtctgtggggtacgtagcctattctcttagccggtatttaaacatacaaattcacccaaattctaccttgataaggtaattgattaatttcataaat

SEQ ID NO: 43 - DNA, 1000 bp, Pichia pastoris
agctcagattggaaatgatttttgatcctaccaagaagcctttgatttccagaatctccgctaagtaagtaacccccgcaaacgcatgcatccatgcaaacaaaatactaacaattttagccccgttgttgagaaacccagaaaattgaatgttcaaccaatccagacgatcaataagaaaaaaggcccaaaggctacttccaaacctgctgccgccaaacctgctccttcaaaagccggtcccaagggaggtaagaaggtgagaaagccaaagaagacagttgaagaattggatcaggaaatggctgactactttgaaaataagaattagcccaacaaaatatgtacaagtattatataaatgaatctacatggtgtgttttatttagatcctccaaaccaaggaaagaaactaaacttatctccggacttacgagtcaaataactatccgcagttccttggaactcagactttcttccataagcggtcatatcatctttggactgtgggaatcctggacgaatctttgaaatgtcataatcttgctctctatctccaagcacagcgtccggtaaatgctggttcttctttctcagatgaatcttggatttaacaaataaagccgtgcctatggctaatgtactcaaaaacaaagtctgcttccagaatttcgcaaacgatggaatgccatttcctgtaaatgtactcattgaacctatgtttgattaaagttggtgtgaagtcatcaaacgagagtaaaatcagatactcgtgcaccggccaaaattgactgagctaatctctgcaggcttgacatccgaacacaacaaataggcgacaaatcttaactatctaatcgtaggctatggtagaactttgtgggggtagaggaagactacaacagcaagacaaaacaaaagagtcatagtttgactctctgcttttttcttctttctcttctttttcttcctccatattcgttatttatttcgaactgga

SEQ ID NO: 44 - DNA, 1000 bp, Pichia pastoris
cagccattaatctcacctcagtttttgaatcagtagaatttttaatgaaacaaacggttggtatattatttgatagagttgccaaatttccaaagataaatttttcatcaggtaatatcctgaataccgtaacatagtgactattggaagacactgctatcatattatatttcggataaaaatccaaaccccagaccgacctcttgagtctcaactccaagtcagccgcaactttaattatccgtggattgggagctagtttggacaacgcatcagtataatataactttacggttccattatcagacgctattgcaagaacttcctttccattgatctcgccaatgcggcagtaattgatatcgtagggtaggtctggaaagacgctggcgcttgtgtcccattctgcaggaatctctggcacggtgctaatggtagttatccaacggagctgaggtagtcgatatatctggatatgccgcctataggataaaaacaggagagggtgaaccttgcttatggctactagattgttcttgtactctgaattctcattatgggaaactaaactaatctcatctgtgtgttgcagtactattgaatcgttgtagtatctacctggagggcattccatgaattagtgagataacagagttgggtaactagagagaataatagacgtatgcatgattactacacaacggatgtcgcactctttccttagttaaaactatcatccaatcacaagatgcgggctggaaagacttgctcccgaaggataatcttctgcttctatctcccttcctcatatggtttcgcagggctcatgccccttcttccttcgaactgcccgatgaggaagtccttagcctatcaaagaattcgggaccatcatcgatttttagagccttacctgatcgcaatcaggatttcactactcatataaatacatcgctcaaagctccaactttgcttgttcatacaattcttgatattcaca

SEQ ID NO: 45 - DNA, 1000 bp, Pichia pastoris
tggttccctctcggtccaataccaaaaatattatcaccatacaggtctcccttcgataccagtgcaaagttgaaccgtgggattaccttggaatctacaaaaatagtgtcactcacaagtttgtcatcaaccacgctgccgcttgcaaaggagaactgaacatgaaggttgttagggtttgttatattggaataagtggtggatttgttgaaggcgaacgcaccaaagctacatccgtcctgagcacactgtgaatttgtcacggaattgaccaagaggtcagacgatcctgtatcccattgagccgttatgctttgtgggggaaaccctatttctatcgtactaagaaaaccaatggtgaactcatattcggtatcaatggcgacgattccagcatagcctgtagacagtaacaacactagggcaacagcaactaacatatcttcattgatgaaacgttgtgatcggtgtgacttttatagtaaaagctacaactgtttgaaataccaagatatcattgtgaatggctcaaaagggtaatacatctgaaaaacctgaagtgtggaaaattccgatggagccaactcatgataacgcagaagtcccattttgccatcttctcttggtatgaaacggtagaaaatgatccgagtatgccaattgatactcttgattcatgccctatagtttgcgtagggtttaattgatctcctggtctatcgatctgggacgcaatgtagaccccattagtggaaacactgaaagggatccaacactctaggcggacccgctcacagtcatttcaggacaatcaccacaggaatcaactacttctcccagtcttccttgcgtgaagcttcaagcctacaacataacacttcttacttaatctttgattctcgaattgtttacccaatcttgacaacttagcctaagcaatactctggggttatatatagcaattgctcttcctcgctgtagcgttcattccatctttcta

SEQ ID NO: 46 - DNA, 1001 bp, Pichia pastoris
gatatcgatctacacttaatagtagatgacgaggcatctctccaataggtaccatatctggtgtttcttgtaatttaagaatctgttggtctatgaatgtagatttgtcatgaacaatgatatatgggtcaggaggacaagatggtttctctgagttgggttgttgaggtgcctggcaagacttcggagcgttgatatccccaagacttgtagtgaccgatagttgaagcgtgtgtttgcaggaacggcacatcaatgcaactttcgtaactttggaattgagagttgatgcactgatgacgatacccgaaattttgacgattttaccaatatgacttgaagacaagtctctcattgaaaccttattatcgttactaagcaaaacgagctgacaagaagggaaggtggtcggtatttcctcgttgttcaaatatatgattctcctggcaatatctgtgatggcctgttcaaaaagtggaatcatttctgcaggatcatctaccaactttttattgagctcctcattgaatacgattaagtggtcattttgaatcgtcagtaagtacttgtttacaagtaaattctgtctgagttgttctctgtagatgtactgattttccatacgaaactccaaaatgaacgaacggaatgccttaatgacctcactgaactggtcatcgttctgttctccgggaaggacacttgtgttaaagactgatgctctatcaaaggacattgcaacaaagtataaacggttgtgagcgggaaaaagatgtgtaggtaattgtcgtagatgagactgattcagtagaaaacgcgtcctgcactatttttttctttcttcattacatttcctaatcgggacaaaatgaatctaaagacgtggttatgtagtacacgcatcgataggctatccccataccaaaacactattttaccccatccttgacaggttataaatatgcgatagtatgagtatcttcaaattcagctgaaatatc

SEQ ID NO: 47 - DNA, 1000 bp, Pichia pastoris
aataaaaaaacgttatagaaagaaattggactacgatatgctccaatccaaattgtcaaaattgaccaccgaaaaagaacaattggaatttgacaagaggaacaactcactagattctcaaacggagcgtcacctagagtcagtttccaagtcaattacagaaagtttggaaacagaagaggagtatctacaattgaattccaaacttaaagtcgagctgtccgaattcatgtcgctaaggctttcttacttggaccccatttttgaaagtttcattaaagttcagtcaaaaattttcatggacatttatgacacattaaagagcggactaccttatgttgattctctatccaaagaggattatcagtccaagatcttggactctagaatagataacattctgtcgaaaatggaagcgctgaaccttcaagcttacattgatgattagagcaatgatataaacaacaattgagtgacaggtctactttgttctcaaaaggccataaccatctgtttgcatctcttatcaccacaccatcctcctcatctggccttcaattgtggggaacaactagcatcccaacaccagactaactccacccagatgaaaccagttgtcgcttaccagtcaatgaatgttgagctaacgttccttgaaactcgaatgatcccagccttgctgcgtatcatccctccgctattccgccgcttgctccaaccatgtttccgcctttttcgaacaagttcaaatacctatctttggcaggacttttcctcctgccttttttagcctcaggtctcggttagcctctaggcaaattctggtcttcatacctatatcaacttttcatcagatagcctttgggttcaaaaaagaactaaagcaggatgcctgatatataaatcccagatgatctgcttttgaaactattttcagtatcttgattcgtttacttacaaacaactattgttgattttatctggagaataatcgaacaaa

SEQ ID NO: 48 - DNA, 1000 bp, Pichia pastoris
attgttgtgaatactctccttcatttggatttcttggacttcggactctcttgatctctcttcgaaagttttaactctgttcatgtataattttacccgctgtaggtcgctcataataccatgagtatgcacatcttttactccattaactttcaggtatgcaaaatacaatgaagatagtatatagctcaaagaatttagcattttgcattgatctaattgtgacattttctctatgatatcatctagcttcttaaactcgagaatctcgtccaacgaggcagaaacattgtccagtcttacgtcaagattattcacgagtttctggaccgtatcaacgttttccatcttaagattacagtaagtatcgtccttttgaactgcaaaggtagaaaagttaatttttgatttggtagtacactatgaaacttgctcaccccaatctttcctcctgacaggttgatctttatccctctactaaattgccccaagtgtatcaagtagactagatctcgcgaaagaacagcctaataaactccgaagcatgatggcctctatccggaaaacgttaagagatgtggcaacaggagggcacatagaatttttaaagacgctgaagaatgctatcatagtccgtaaaaatgtgatagtactttgtttagtgcgtacgccacttattcggggccaatagctaaacccaggtttgctggcagcaaattcaactgtagattgaatctctctaacaataatggtgttcaatcccctggctggtcacggggaggactatcttgcgtgatccgcttggaaaatgttgtgtatccctttctcaattgcggaaagcatctgctacttcccataggcaccagttacccaattgatatttccaaaaaagattaccatatgttcatctagaagtataaatacaagtggacattcaatgaatatttcattcaattagtcattgacactttcatcaacttactacgtcttattcaacaat

SEQ ID NO: 49 - DNA, 1000 bp, Pichia pastoris
tatacggtctatccactttggaaacgatgtagttgaaacggggaagtaatagtggttcccaaacgacatgaagaggttatataagtttgcaagagggtgacaccattttagttgtggttcccgggtatttttttaatctttttagtctaagatagcctccccagatattaccgagttgggccatttggggcggtatcggtggtatctgatggtagcgcgtttttacatgcctgtgcattgaactggcaaagagtatactatcgtggggccctgaaggaggcagcaaatggaccgtcaattggttgatcagggactcaagacaggtattgagcttttcaaacaaaaagagtataggcgctgctacaaggcatttacttctactatcaatttcattgagaatgatcccgagttggccgccagctgtgtatctcaactgatatctctgttagattgtagggcagcctgtttggaaaagctagatcaattgaatatggccttgaaagatggtcttaaaatgatcaagagagagtgccacaactgcaagggttatttgagaacttgcaaaattttagacctacaagggaagatcagtgaggctttgtctacagcaagagaagggatctccataatagaaactagaagagatcaggataatcaatttagatattccaaggttcttttggaacaattaaaggaactgaaaaatgcactgaaaatcaaattggacaagaaaaatcagctacacttcaaagttttaaagtttgacgcaccagtgccttgtacaaagaaactaagattagtcactccaagaacaatagatccttccatttttttgccgatagagctagtgaagctgatctttcgcctgttgaatttctcagacatgtatgcctgtttattggtctcaacaaaatggaactcaattatatcctcatcaccggaactgtttcgaaaacttcagttgaaatcccaactgtccaacaaggcgttaaacaattgt

SEQ ID NO: 50 - protein, 350 aa, Komagataella phaffii
MSPTIPTTQKAVIFETNGGPLEYKDIPVPKPKSNELLINVKYSGVCHTDLHAWKGDWPLDNKLPLVGGHEGAGVVVAYGENVTGWEIGDYAGIKWLNGSCLNCEYCIQGAESSCAKADLSGFTHDGSFQQYATADATQAARIPKEADLAEVAPILCAGITVYKALKTADLRIGQWVAISGAGGGLGSLAVQYAKALGLRVLGIDGGADKGEFVKSLGAEVFVDFTKTKDVVAEVQKLTNGGPHGVINVSVSPHAINQSVQYVRTLGKVVLVGLPSGAVVNSDVFWHVLKSIEIKGSYVGNREDSAEAIDLFTRGLVKAPIKIIGLSELAKVYEQMEAGAIIGRYVVDTSK

SEQ ID NO: 51 - DNA, 1053 bp, Komagataella phaffii
atgtctccaactatcccaactacacaaaaggctgttatcttcgagaccaacggcggtcccctagagtacaaggacattccagtcccaaagccaaagtcaaacgaacttttgatcaacgttaagtactccggtgtctgtcacactgatttgcacgcctggaagggtgactggccattggacaacaagcttcctttggttggtggtcacgaaggtgctggtgtcgttgtcgcttacggtgagaacgtcactggatgggagatcggtgactacgctggtatcaaatggttgaacggttcttgtttgaactgtgagtactgtatccaaggtgctgaatccagttgtgccaaggctgacctgtctggtttcacccacgacggatctttccagcagtatgctactgctgatgccacccaagccgccagaattccaaaggaggctgacttggctgaagttgccccaattctgtgtgctggtatcaccgtttacaaggctcttaagaccgctgacttgcgtattggccaatgggttgccatttctggtgctggtggaggactgggttctcttgccgttcaatacgccaaggctctgggtttgagagttttgggtattgatggtggtgccgacaagggtgaatttgtcaagtccttgggtgctgaggtcttcgtcgacttcactaagactaaggacgtcgttgctgaagtccaaaagctcaccaacggtggtccacacggtgttattaacgtctccgtttccccacatgctatcaaccaatctgtccaatacgttagaactttgggtaaggttgttttggttggtctgccatctggtgccgttgtcaactctgacgttttctggcacgttctgaagtccatcgagatcaagggatcttacgttggaaacagagaggacagtgccgaggccatcgacttgttcaccagaggtttggtcaaggctcctatcaagattatcggtctgtctgaacttgctaaggtctacgaacagatggaggctggtgccatcatcggtagatacgttgtggacacttccaaataa

SEQ ID NO: 52 - protein, 350 aa, Komagataella pastoris
MSPTIPSTQKAVVFETNGGPLEYKDIPVPKPKSNEILINVKYSGVCHTDLHAWKGDWPLDNKLPLVGGHEGAGVVVALGENVTGWNIGDYAGIKWLNGSCLNCEYCIQGAESSCAKADLSGFTHDGSFQQYATADATQAARIPKEVDLAEVAPILCAGITVYKALKTADLRIGQWVAISGAGGGLGSLAVQYAKALGLRVLGIDGGADKGEFVKSLGAEVYVDFTKTKDVVAEVQKATNGGPHGVINVSVSPHAINQSVQYARTLGKIVLVGLPSGAVVNSDVFWHVLKSIEIKGSYVGNREDSAEAIDLFARGLVKAPIKIIGLSELAKVYEQMEAGAIIGRYVVDTSK

SEQ ID NO: 53 - DNA, 1053 bp, Komagataella pastoris
atgtctccaactatcccatctacacaaaaggctgttgtcttcgagaccaacggcggtcctctcgagtacaaggacatccctgtcccaaagccaaagtccaacgaaatcttgatcaacgttaagtactccggtgtctgtcacactgacttgcacgcctggaagggtgactggccattggacaacaagcttcctttggtcggtggtcacgaaggtgctggtgtcgttgtcgctttaggtgagaacgtcactggatggaacatcggtgactacgctggtatcaaatggttgaacggttcttgtttgaactgtgagtactgtatccaaggtgctgaatccagttgtgccaaggctgacctgtctggtttcacccacgacggatctttccagcagtatgctactgctgatgccacccaagccgccagaattccaaaggaagttgacttggctgaagttgccccaattttgtgtgctggtatcaccgtttacaaggctcttaagaccgctgacttgcgtatcggccaatgggttgccatttccggtgctggtggaggattaggttctcttgccgttcaatacgccaaggctctgggtttgagagttttgggtattgatggtggtgccgacaagggtgagttcgtcaagtccttgggtgctgaggtctacgtcgacttcactaagactaaggacgtcgttgctgaggtccaaaaggccaccaacggtggtccacacggtgttatcaacgtctccgtttccccacatgctatcaaccaatctgtccaatacgctagaactttgggtaagattgttttggttggtctgccatctggtgccgttgtcaactctgacgttttctggcacgttctgaagtccatcgagatcaagggatcttacgttggaaacagagaggacagtgccgaagccatcgacttgttcgctagaggcttagtcaaggctcctattaagattattggtctgtccgaacttgctaaggtctacgagcagatggaggctggtgccatcatcggtagatacgttgtggacacttccaaataa

SEQ ID NO: 54 - protein, 349 aa, Ogataea parapolymorpha
MTSIPKTQKAVVFETNGGPLLYKDIPVPQPKPNEILVNVKYSGVCHTDLHAWKGDWPLDTKLPLVGGHEGAGVVVAKGANVTNFEIGDYAGIKWLNGSCMGCEFCQQGAEPNCPEADLSGYTHDGSFQQYATADAVQAAKIPKGTNLADVAPILCAGVTVYKALKTAELSPGQWVAISGAGGGLGSLAVQYAVAMGLRVLGIDGGDEKAKLFESLGGEVFIDFTKEKDIVGAVQKATNGGPHGVINVSVSPAAISQSCQYVRTLGKVVLVGLPAGAVCESPVFEHVIKSIQIRGSYVGNRQDTAESIDFFVRGKVKAPIKVVGLSELPKVFELMEQGKIAGRYVLDTSK

SEQ ID NO: 55 - DNA, 1050 bp, Ogataea parapolymorpha
atgacttccattccaaagactcaaaaggccgttgttttcgagaccaacggtggtcctcttctctacaaggacatccctgttccacaaccaaagccaaatgagattcttgtcaacgtcaagtactccggtgtttgccacaccgatctccacgcttggaagggtgactggccattggacaccaaacttccactggtcggtggtcacgagggtgctggtgttgttgttgctaagggtgccaacgttaccaactttgaaatcggtgactacgctggtatcaaatggttgaacggctcgtgcatgggttgtgagttctgtcaacaaggtgcagagccaaactgtcctgaggccgacctttccggttacacgcacgacggttctttccaacaatacgccactgctgatgctgtccaggctgccaagattccaaagggaactaacctggctgacgttgctccaattctctgtgctggtgtcactgtgtacaaggcattgaagactgccgaattgagcccaggccaatgggttgctatctctggtgctggtggaggattgggttctcttgccgttcaatacgctgtcgccatgggcctgagagtcctgggtatcgatggtggtgacgaaaaggctaagctcttcgagagcttgggcggagaagtcttcatcgatttcaccaaggaaaaggacattgtcggagccgtccagaaggcaaccaacggtggtccacacggtgttatcaacgtttctgtgtctccagcagctatctctcaatcctgccaatacgtgagaactcttggtaaggttgttcttgttggtcttccagccggtgctgtttgcgagtctccagttttcgagcacgttatcaagtctatccagattagaggttcctacgttggtaacagacaggacactgccgagtcgattgacttcttcgtcagaggcaaggttaaggctccaatcaaggttgttggcctttctgagctgccaaaggtgttcgagttgatggagcaaggaaagattgctggaagatacgttcttgacacttccaaatag

SEQ ID NO: 56 - protein, 382 aa, Ogataea parapolymorpha
MMSISRVAALRNQFARLAKPAVVQQVFRHSTASAPTIPKTQMGCVFETNGGPIEYKEIPVPKPKPNEILVHVKYSGVCHTDLHAWKGDWPLPVKLPLVGGHEGAGVVVAKGENVKNFEIGDLAGIKWLNGSCMGCEFCQQGAEPNCPDADLSGYTHDGSFQQYATADAVQAAKLPPGTDLAAVAPILCAGVTVYKALKTAALRPGQIVAISGAAGGLGSLAVQYAVAMGLRVLGIDGGEQKGEFIKKLGAEFYVDFTKEKDIVSAIQKITNGGPHGVINVSVSPAAISQSCQYVRTLGKVVLVGLPAGAVCESPVFEHVVKSIQIKGSYVGNRQDTAEAVDFFTRGLVKSPFQIAGLSELPEVFKKMEEGKILGRYVLDTSK

SEQ ID NO: 57 - DNA, 1149 bp, Ogataea parapolymorpha
atgatgtctatttcgagagttgctgctttgagaaaccaatttgctcggctagccaagcccgctgttgtccagcaggtcttcagacactctactgcctctgctccaaccatcccaaagacccagatgggatgtgtttttgaaaccaacggtggtccaattgagtacaaggagatccctgttccaaagccaaagcctaacgagattttggtccacgtcaagtactctggtgtgtgccacactgacttgcacgcctggaagggtgactggccactgcctgtcaaactcccacttgtgggtggtcacgagggtgccggtgttgtcgttgccaagggtgagaacgttaaaaacttcgagatcggcgacttggccggtatcaagtggctgaacggctcgtgtatgggttgtgagttctgtcaacagggtgccgaaccaaactgtccagacgctgacctgtccggttacacgcacgacggttctttccaacaatacgccactgctgacgctgtccaggccgctaagctgcctcctggaactgacctcgctgctgttgctcctattttgtgtgctggtgtcactgtttacaaggccttgaagactgctgctctgcgtccaggacagatcgttgccatttccggtgccgccggtggattgggttctcttgccgttcaatacgctgtcgccatgggcctgagagttctgggtattgacggtggtgagcaaaagggcgagttcatcaagaagctcggtgccgaattctacgtcgacttcaccaaggagaaggacattgtgtctgccatccagaagatcaccaacggcggtccacacggtgtcatcaacgtttctgtctctccagctgctatctcccagtcttgtcaatacgtgagaaccctcggtaaggttgttctggtcggtcttccagccggcgctgtttgcgagtctcctgtctttgagcacgtcgtcaagtccatccagatcaagggatcttacgttggtaacagacaagacactgccgaggccgtggacttcttcaccagaggccttgtcaagtctccattccagattgctggtctttccgagctgccagaggtcttcaagaagatggaggagggcaagatcttgggcagatacgtccttgacacttctaaatag

SEQ ID NO: 58 - protein, 349 aa, Ogataea polymorpha
MPSIPKTQKAIVFETNGGPLLYKDIPVPQPKPNEILVNVKYSGVCHTDLHAWKGDWPLATKLPLVGGHEGAGVVVAKGANVTNFEIGDYAGIKWLNGSCMGCEFCQQGAEPNCPDADLSGYTHDGSFQQYATADAVQAAKIPKGTNLADVAPILCAGVTVYKALKTAELSPGQWVAISGAGGGLGSLAVQYAVAMGLRVLGIDGGDEKAKLFESLGGEVFIDFTKEKDIVGAVQKATNGGPHGVINVSVSPAAISQSCQYVRTLGKVVLVGLPAGAVCESPVFEHVIKSIQIRGSYVGNRQDTAESIDFFVRGKVKAPIKVVGLSELPKVFELMEQGKIAGRYVLDTSK

SEQ ID NO: 59 - DNA, 1050 bp, Ogataea polymorpha
atgccttccattccaaagactcaaaaggccattgttttcgaaaccaacggtggtcctcttctatacaaggacatccctgttccacagccaaagccaaatgaaatccttgtcaacgtcaagtactctggtgtgtgccacaccgacttgcacgcctggaagggtgactggccattggccaccaaacttccactggtcggtggtcacgagggtgctggtgttgttgttgccaagggtgccaacgttaccaactttgagatcggcgactacgctggtatcaaatggctgaacggctcgtgtatgggttgtgagttctgtcaacaaggtgcagaaccaaactgtccagacgccgacctttccggttacacgcacgacggttccttccaacaatacgccactgctgatgctgtccaggctgccaagattccaaagggaactaacctggccgatgttgctccaattctctgtgctggtgtcactgtgtacaaggcattgaagactgccgaattgagcccaggccagtgggtcgctatctctggtgctggtggaggattgggttctcttgccgttcaatacgctgtcgctatgggcctgagagttctgggtatcgatggtggtgacgaaaaggccaagctcttcgagagcttgggcggagaagtcttcatcgatttcacaaaggaaaaggacattgtcggagccgtccagaaggctaccaacggtggtccacacggtgtcatcaacgtttccgtgtctccagcagctatctctcaatcctgccaatacgtgagaactcttggtaaggttgttcttgttggtcttccagcaggtgctgtttgcgagtctccagttttcgagcacgttatcaagtctatccagattagaggttcctacgttggtaacagacaggacactgcggagtcgatcgacttcttcgtcagaggcaaggttaaggctccaatcaaggttgttggtctttctgagctgccaaaagtgttcgagttgatggagcaaggaaagattgcaggaagatacgtcctcgacacttccaaatag

SEQ ID NO: 60 - protein, 381 aa, Ogataea polymorpha
MSISRVAALRNQFARLAKPAVVQQVFRHSTASAPTIPKTQMGCVFETNGGPIEYKEIPVPKPKPNEILVHVKYSGVCHTDLHAWKGDWPLPVKLPLVGGHEGAGVVVAKGENVKNFEIGDLAGIKWLNGSCMGCEFCQQGAEPNCPDADLSGYTHDGSFQQYATADAVQAAKLPPGTDLAAVAPILCAGVTVYKALKTAALRPGQIVAISGAAGGLGSLAVQYAVAMGLRVLGIDGGEQKGEFIKKLGAEFYVDFTKEKDIVSAIQKVTNGGPHGVINVSVSPAAISQSCQYVRTLGKVVLVGLPAGAVCESPVFEHVVKSIQIKGSYVGNRQDTAEAVDFFTRGLVRSPFQIAGLSELPEVFKKMEEGKILGRYVLDTSK

SEQ ID NO: 61 - DNA, 1146 bp, Ogataea polymorpha
atgtctatttcgagagttgctgcattgagaaaccaatttgctcgtctagccaagccggctgtagtccagcaggtcttcagacactccactgcctctgctccaaccatcccaaagacccagatgggatgtgtttttgaaaccaacggcggtccaattgagtacaaggagatcccagttccaaagccaaagccaaacgagattctggtccacgtcaagtactctggtgtgtgccacaccgacttgcacgcctggaagggtgactggccactgcctgtcaaactcccacttgtgggtggtcacgagggtgccggtgttgtcgttgccaagggtgagaacgttaaaaacttcgagatcggcgacttggccggtatcaaatggctgaacggctcgtgtatgggttgtgagttctgtcaacagggtgccgaaccaaactgtcctgacgccgacctttccggttacacacacgacggttctttccaacaatacgccactgctgacgctgtccaggccgctaagctgcctccaggaactgacctcgctgctgttgctccaattttgtgtgctggtgtgactgtttacaaggccttgaagactgctgctttgcgtccaggtcagattgttgctatttccggtgccgccggtggattgggttctcttgccgttcaatacgctgtcgccatgggtctgagagttctgggtattgacggtggtgagcagaagggcgagttcatcaagaagctcggtgccgaattctacgtcgacttcaccaaggagaaggacattgtgtctgccatccagaaggtcaccaatggcggtccacacggtgtcatcaacgtgtctgtgtctccagctgctatctcccagtcttgtcaatacgtgagaaccctcggtaaggttgttctggttggtcttccagccggcgctgtttgcgaatctcctgtctttgagcacgtcgtcaagtccatccagatcaagggatcttatgttggtaacagacaagacactgccgaggccgtggacttcttcaccagaggccttgtccgttctccattccaaattgccggtctttccgagctgcctgaggtcttcaagaagatggaggagggcaagatcttgggtagatatgtccttgacacttctaaataa

SEQ ID NO: 62 - protein, 348 aa, Saccharomyces cerevisiae
MSIPETQKAIIFYESNGKLEYKDIPVPKPKANELLINVKYSGVCHTDLHAWHGDWPLPVKLPLVGGHEGAGVVVGMGENVKGWKIGDYAGIKWLNGSCMACEYCELGNESNCPHADLSGYTHDGSFQQYATADAVQAAHIPQGTDLAEVAPVLCAGITVYKALKSANLRAGHWVAISGAAGGLGSLAVQYAKAMGYRVLGIDGGPGKEELFTSLGGEVFIDFTKEKDIVSAVVKATNGGAHGIINVSVSEAAIEASTRYCRANGTVVLVGLPAGAKCSSDVFNHVVKSISIVGSYVGNRADTREALDFFARGLVKSPIKVVGLSSLPEIYEKMEKGQIAGRYVVDTSK

SEQ ID NO: 63 - DNA, 1047 bp, Saccharomyces cerevisiae
atgtctattccagaaactcaaaaagccattatcttctacgagtccaacggtaagttggaatacaaagatattccagttccaaagccaaaggccaacgaattgttgatcaacgttaaatactctggtgtctgtcacactgacttgcacgcttggcacggtgactggccattgccagttaagctaccattagtcggtggtcacgaaggtgccggtgtcgttgtcggcatgggtgaaaacgttaagggctggaagatcggtgactacgccggtatcaaatggttgaacggttcttgtatggcctgtgaatactgtgaattgggtaacgaatccaactgtcctcacgctgacttgtctggttacacccacgacggttctttccaacaatacgctaccgctgacgctgttcaagccgctcacattcctcaaggtactgacttggctgaagtcgccccagttttgtgtgctggtatcaccgtctacaaggctttgaagtctgccaacttgagagcaggccactgggtggccatttctggtgctgctggtggtctaggttctttggctgttcaatatgctaaggcgatgggttacagagtcttaggtattgatggtggtccaggaaaggaagaattgtttacctcgctcggtggtgaagtattcatcgacttcaccaaagagaaggacattgttagcgcagtcgttaaggctaccaacggcggtgcccacggtatcatcaatgtttccgtttccgaagccgctatcgaagcttctaccagatactgtagggcgaacggtactgttgtcttggttggtttgccagccggtgcaaagtgctcctctgatgtcttcaaccacgttgtcaagtctatctccattgtcggctcttacgtggggaacagagctgataccagagaagccttagatttctttgccagaggtctagtcaagtctccaataaaggtagttggcttatccagtttaccagaaatttacgaaaagatggagaagggccaaattgctggtagatacgttgttgacacttctaaataa

SEQ ID NO: 64 - protein, 349 aa, Candida maltosa
MSSIPTTQKAIIFETNGGKLEYKDIPVPKPKPNELLINVKYSGVCHTDLHAWKGDWPLATKLPLVGGHEGAGVVVAIGDNVKNWKVGDFAGVKWLNGSCLNCEYCQQGAEPNCAQADLSGYTHDGSFQQYATADAVQAARIPAGTDLATVAPILCAGVTVYKALKTANLQPGQWVAISGAAGGLGSLAVQYAKAMGYRVLAIDGGEDKGQFVKSLGAETFIDFTKEKDVVGAVQKATNGGPHGVINVSVSDRAINQSVEYVRTLGKVVLVGLPAGAKVTAPVFDSVVKSIEIKGSYVGNRKDTAEAVDFFSRGLIKCPIKIVGLSELPEVYKLMEEGKILGRYVLDTSK

SEQ ID NO: 65 - DNA, 1050 bp, Candida maltosa
atgtcttctattccaactactcaaaaagctattatcttcgaaaccaacggcggtaaattagaatacaaagatatcccagtcccaaaaccaaaaccaaatgaattgttgatcaatgttaaatactccggtgtttgtcacactgatttgcacgcttggaaaggtgattggccattagccaccaaattaccattggtcggtggtcacgaaggtgctggtgttgtcgttgctattggtgacaatgtcaagaactggaaagttggtgatttcgccggtgtcaaatggttgaatggttcttgtttgaactgtgaatactgtcaacaaggtgctgaaccaaactgtgctcaagctgacttgtccggttacacccacgatggttctttccaacaatacgccactgccgatgcagttcaagcggctagaattccagctggtactgatttagccaccgttgctccaatcttgtgtgctggtgttaccgtttacaaggctttgaagactgccaacttacaaccaggtcaatgggttgccatttccggtgccgctggtggtttaggttctttggctgttcaatacgctaaagctatgggttacagagtcttggccattgacggtggtgaagataaaggtcaatttgttaaatctttgggtgctgaaacttttatcgattttaccaaagaaaaggatgttgttggtgctgtccaaaaagctaccaacggtggtccacatggtgtcattaacgtctctgtttccgacagagctatcaaccaatccgttgaatacgttagaactttaggtaaagttgttttggttggtttaccagctggtgctaaagtcactgctccagtctttgactccgtcgttaaatccattgaaattaaaggttcttatgttggtaacagaaaagacactgccgaagccgttgatttcttctctagaggtttgattaaatgtccaatcaagattgttggtttatctgaattaccagaagtttacaaattgatggaagaaggtaaaatcttgggtagatacgttttggacacctccaaataa

SEQ ID NO: 66 - protein, 379 aa, Kluyveromyces marxianus
MFRLARAQTSITTTSKALGGSRRLFVRLNSSFAIPESQKGVIFYENGGKLEYKDLPVPKPKPNEILINVKYSGVCHTDLHAWKGDWPLPVKLPLVGGHEGAGVVVAKGENVTNFEIGDYAGIKWLNGSCMSCELCEQGYESNCLQADLSGYTHDGSFQQYATADAVQAAQIPKGTDLAEIAPILCAGVTVYKALKTADLQPGQWIAISGAAGGLGSLAVQYAKAMGLRVLGIDGGPGKEELFKSLGGEVFIDFTKSKDMVADIQEATNGGPHGVINVSVSEAAISMSTEYVRPTGVVVLVGLPAHAYVKSEVFSHVVKSISIKGSYVGNRADTREAIDFFTRGLVKSPIKVVGLSELPKVYELMEAGKILGRYVVDTSK

SEQ ID NO: 67 - DNA, 1140 bp, Kluyveromyces marxianus
atgttcagactagcacgcgctcagaccagcattaccaccactagcaaggctctaggtggctccagaagactattcgtcagactaaactcctctttcgccatcccagaatcccaaaagggtgtgattttctacgaaaacggcggtaagttggaatacaaggaccttccagttccaaagccaaagccaaatgaaatcttgatcaacgtcaagtactccggtgtgtgtcacactgatttgcacgcctggaagggtgactggccattgccagttaagttgcctttggtcggtggtcacgaaggtgccggtgtcgtcgttgccaagggtgaaaacgttaccaacttcgagatcggtgactacgcaggtatcaagtggttgaacggttcttgtatgtcttgtgaactctgtgaacaaggttacgaatccaactgtttgcaagctgacttgtctggttacacccacgacggttccttccaacaatatgccactgctgacgctgttcaagctgcccaaattccaaagggtaccgatttggctgaaatcgccccaatcttgtgtgccggtgtcaccgtctacaaggctctaaagaccgctgacttgcaaccaggtcaatggatcgctatctccggtgctgccggtggtcttggttccctagccgtgcaatacgccaaggcaatgggtctaagagttctaggtatcgacggtggtccaggtaaggaagaattgttcaagagcttgggtggtgaagtcttcattgacttcacaaagtccaaggacatggtcgcagacatccaggaagccaccaacggtggtcctcacggtgtgatcaacgtctccgtctccgaggccgctatctccatgtccaccgagtacgtcagaccaaccggtgtggtcgttctagtcggtttgccagcccacgcttacgtcaagtccgaagtcttctcccacgtcgtcaagtctatctctattaagggttcttacgtcggtaacagagcagacaccagagaagctattgacttcttcaccagaggtttggtcaagtctccaatcaaggttgttggtttgtctgaattgccaaaggtttatgaattgatggaagctggtaagatcttgggtagatacgtcgttgacacttccaaataa

SEQ ID NO: 68 - protein, 350 aa, Escherichia coli
MSEQIPKTQKAVVFDTNGGQLVYKDYPVPTPKPNELLINVKYSGVCHTDLHAWKGDWPLATKLPLVGGHEGAGVVVGMGENVKGWKIGDFAGIKWLNGSCMSCEFCQQGAEPNCGEADLSGYTHDGSFEQYATADAVQAAKIPAGTDLANVAPILCAGVTVYKALKTADLAAGQWVAISGAGGGLGSLAVQYARAMGLRVVAIDGGDEKGEFVKSLGAEAYVDFTKDKDIVEAVKKATDGGPHGAINVSVSEKAIDQSVEYVRPLGKVVLVGLPAHAKVTAPVFDAVVKSIEIKGSYVGNRKDTAEAIDFFSRGLIKCPIKIVGLSDLPEVFKLMEEGKILGRYVLDTSK

SEQ ID NO: 69 - DNA, 1053 bp, Escherichia coli
atgtctgaacaaatcccaaaaactcaaaaagccgttgtctttgataccaatggtggtcaattagtctacaaggattacccagttccaactccaaagccaaatgaattgttaatcaacgtcaaatactctggtgtctgtcacactgatttacacgcttggaaaggtgactggccattggctactaaattgccattagttggtggtcacgaaggtgccggtgtcgttgtcggtatgggtgaaaacgtcaaaggatggaaaatcggtgactttgccggtatcaaatggttgaacggttcttgtatgagttgtgaattctgtcaacaaggtgctgaaccaaactgtggtgaagctgacttgtctggttacactcacgatggttcattcgaacaatacgctactgctgatgctgtccaagccgctaaaattccagctggtactgatttagccaatgtcgcaccaatcttatgtgctggtgttactgtttacaaagccttaaagactgctgacttagcagctggccaatgggttgctatctccggtgctggtggtggtttaggttctttggccgttcaatacgccagagccatgggtttgagagttgttgctattgacggtggtgacgaaaaaggtgaatttgttaaatcattgggtgctgaagcttacgttgatttcaccaaagataaagatattgttgaagctgttaagaaggctactgatggtggtccacacggtgctatcaatgtctctgtttctgaaaaagccattgaccaatctgttgaatatgttagaccattaggtaaagttgttttggttggtttaccagctcacgctaaagtcactgctccagttttcgatgctgttgtcaaatccattgaaatcaaaggttcttacgttggtaacagaaaagatactgctgaagctattgacttcttctccagaggtttaatcaaatgcccaatcaagattgtcggtttatctgacttgccagaagtcttcaaattgatggaagaaggtaaaatcttgggtagatacgtcttggacaccagtaaataa

SEQ ID NO: 70 - protein, 353 aa, Fusarium graminearum
MAAPQIPSQQWAQIFEKTAGPIEYKQIPVQKPGPDEVLVNVKFSGVCHTDLHAWQGDWPLDTKLPLVGGHEGAGVVVARGELVKDVKIGEKVGIKWLNGSCLSCSYCQNADESLCAEALLSGYTVDGSFQQYAIAKAIHVARIPEECDLEAISPILCAGITVYKGIKESGVKAGQSLAIVGAGGGLGSIAVQYAKAMGIHAIAIDGGEEKEKMCMSLGAQTFIDFTKTKNIVADVKATTNDGLGPHAALLVAAAEKPFQQATQYIRSKGTVVCIGLPAGAQFSAPVFDTVVRMIQIKGSYVGNRADTAEAIDFFRRGLIKVPFKTVGLSELNEVFKLMKAGQVAGRYVVDTSR

SEQ ID NO: 71 - DNA, 1062 bp, Fusarium graminearum
atggccgctccccagattccttcccagcagtgggctcagatcttcgagaagaccgccggtcccatcgagtacaagcagattcccgtccagaagcctggccccgatgaggttctcgtcaacgtcaagttctccggtgtctgccacactgacctccacgcctggcagggtgactggcccctcgacaccaagctgccccttgtcggtggccacgagggtgccggtgttgtcgttgcccgcggcgagcttgtcaaggatgtcaagattggcgagaaggtcggtatcaagtggctcaacggttcttgcttgagctgctcttactgccaaaacgccgatgagtctctctgcgctgaggctcttctctccggttacaccgtcgatggatctttccagcaatacgccatcgccaaggctatccacgttgctcgcatccctgaggagtgtgaccttgaggccatctcccccattctctgcgccggtatcaccgtctacaagggtatcaaggagtccggtgtcaaggccggccagtctcttgctatcgtcggtgctggtggtggtctcggttccatcgctgttcagtacgccaaggctatgggtatccatgccattgccattgatggtggtgaggagaaggagaagatgtgcatgtctctcggtgcccaaaccttcatcgacttcacaaagactaagaacatcgtcgctgatgtcaaggctactaccaacgatggccttggccctcacgctgctctcctcgtcgctgctgccgagaagcccttccaacaggctacccaatacatccgatccaagggtaccgtcgtctgcatcggtctccccgctggtgctcagttctctgcccccgtcttcgacactgtcgttcgcatgattcagatcaagggatcttatgtcggtaaccgtgccgatactgctgaggccatcgacttcttccgccgtggtctcatcaaggttcccttcaagactgttggtctctctgagctcaacgaggtcttcaagctcatgaaggctggccaagttgctggtcgctatgtcgttgacaccagccgataa

SEQ ID NO: 72 - DNA, 1966 bp, Artificial Sequence
  Adh2 split marker cassette 1
cgtatctaccgatgatggcaccagcctccatctgttcgtagaccttagcaagttcagacagaccgataatcttgataggagccttgaccaaacctctggtgaacaagtcgatggcctcggcactgtcctctctgtttccaacgtaagatcccttgatctcgatggacttcagaacgtgccagaaaacgtcagagttgacaacggcaccagatggcagaccaaccaaaacaaccttacccaaagttctaacgtattggacagattggttgatagcatgtggggaaacggagacgttaataacaccgtgtggaccaccgttggtgagcttttggacttcagcaacgacgtccttagtcttagtgaagtcgacgaagacctcagcacccaaggacttgacaaattcacccttgtcggcaccaccatcaatacccaaaactctcaaacccagagccttggcgtattgaacggcaagagaacccagtcctccaccagcaccagaaatggcaacccattggccaatacgcaagtcagcggtcttaagagccttgtaaacggtgataccagcacacagaattggggcaacttcagccaagtcagcctcctttggaattctggcggcttgggtggcatcagcagtagcatactgctggaaagatccgtcgtgggtgaaaccagacaggtcagccttggcacaactggattcagcaccttggatacagtactcacagttcaaacaagaaccgttcaaccatttgataccagcgtagtcaccgatagtggatctgatatcacctaataacttcgtatagcatacattatacgaagttatattaagggttctcgaatggtaccttgctcacatgttgatctccagcttgcaaattaaagccttcgagcgtcccaaaaccttctcaagcaaggttttcagtataatgttacatgcgtacacgcgtctgtacagaaaaaaaagaaaaatttgaaatataaataacgttcttaatactaacataactataaaaaaataaatagggacctagacttcaggttgtctaactccttccttttcggttagagcggatgtggggggagggcgtgaatgtaagcgtgacataactaattacatgatatcgacaaaggaaaagggggacggatctccgaggtaaaatagaacaactacaatataaaaaaactatacaaatgacaagttcttgaaaacaagaatctttttattgtcagtactgattattcctttgccctcggacgagtgctggggcgtcggtttccactatcggcgagtacttctacacagccatcggtccagacggccgcgcttctgcgggcgatttgtgtacgcccgacagtcccggctccggatcggacgattgcgtcgcatcgaccctgcgcccaagctgcatcatcgaaattgccgtcaaccaagctctgatagagttggtcaagaccaatgcggagcatatacgcccggagccgcggcgatcctgcaagctccggatgcctccgctcgaagtagcgcgtctgctgctccatacaagccaaccacggcctccagaagaagatgttggcgacctcgtattgggaatccccgaacatcgcctcgctccagtcaatgaccgctgttatgcggccattgtccgtcaggacattgttggagccgaaatccgcgtgcacgaggtgccggacttcggggcagtcctcggcccaaagcatcagctcatcgagagcctgcgcgacggacgcactgacggtgtcgtccatcacagtttgccagtgatacacatggggatcagcaatcgcgcatatgaaatcacgccatgtagtgtattgaccgattccttgcggtccgaatgggccgaacccgctcgtctggctaagatcggccgcagcgatcgcatccatggcctccgcgaccggctgcagaacagcgggcagttcggtttcaggcaggtct

SEQ ID NO: 73 - DNA, 2069 bp, Artificial Sequence
  Adh2 split marker cassette 2
  misc_feature (1099)..(1099): n is a, c, g, or t
agatgttggcgacctcgtattgggaatccccgaacatcgcctcgctccagtcaatgaccgctgttatgcggccattgtccgtcaggacattgttggagccgaaatccgcgtgcacgaggtgccggacttcggggcagtcctcggcccaaagcatcagctcatcgagagcctgcgcgacggacgcactgacggtgtcgtccatcacagtttgccagtgatacacatggggatcagcaatcgcgcatatgaaatcacgccatgtagtgtattgaccgattccttgcggtccgaatgggccgaacccgctcgtctggctaagatcggccgcagcgatcgcatccatggcctccgcgaccggctgcagaacagcgggcagttcggtttcaggcaggtcttgcaacgtgacaccctgtgcacggcgggagatgcaataggtcaggctctcgctgaattccccaatgtcaagcacttccggaatcgggagcgcggccgatgcaaagtgccgataaacataacgatctttgtagaaaccatcggcgcagctatttacccgcaggacatatccacgccctcctacatcgaagctgaaagcacgagattcttcgccctccgagagctgcatcaggtcggagacgctgtcgaacttttcgatcagaaacttctcgacagacgtcgcggtgagttcaggctttttacccatggtttagttcctcaccttgtcgtattatactatgccgatatactatgccgatgattaattgtcaacaccgcccttagattagattgctatgctttctttctaatgagcaagaagtaaaaaaagttgtaatagaacaagaaaaatgaaactgaaacttgagaaattgaagaccgtttattaacttaaatatcaatgggaggtcatcgaaagagaaaaaaatcaaaaaaaaaaaattttcaagaaaaagaaacgtgataaaaatttttattgcctttttagacgaagaaaaagaaacgaggcggtctcttttttcttttccaaacctttagtacgggtaattaacgacaccctagaggaagaaagaggggaaatttagtatgctgtgcttgggggttttgnaaatggtacggcgatgcgcggaatccgagaaaatctggaagagtaaaaaaggagtagaaacattttgaagctatggtgtgtggtaccgatctagacctaataacttcgtatagcatacattatacgaagttatattaagggttgtcgacctgcagcgtacggcacgaattcgcaccccggagagcgctcacccccgttttcaaacagcggggggagcacaaaatgttgaaaactacacagatcttttcggacaccggtcgctttatgtagtcgacatgcagattctcccaaatggaaaacgagattggacaatttgtggagttggaaaggggggtgggaatcaacgaaattagcagattcatgggcaattggcaggactgggcagaaggggtgagaattgcaatcgaatggaacaggcactcccgttgcgaaatcaaaaaagtctcgctatctgaactgattttttttaagcagcaacttacggtcaatacatctccgatggaggaatttttcacccctcgctaactagatgggccccttctaagaaatttgggtttaaggttgggcagtcagtcagtgcaccaatgctaactgccatttgtccaaagaggggtgcaaggatgagggaccgttgagaataagatttggggtgttaatcggtgatactgatttgtcaaagagtggggaggactgctgggcattgttcacccccctagttgttagagttcgatagccggccgaatcacccccctcttcttacataatcattgtcactatgtggggtctctacagtctcaccctgcgatccgggacgacgccgcgaaattagggggcaagtctcctccgggcatgcaatattggtaacaggatcaattgatgcgagaaaagttggagggggtgtaaaattcaagcccacaaagtcacacccttatgcctgtagaggggcaatcggagagcagccatggggtgt

SEQ ID NO: 74 - DNA, 1850 bp, Artificial Sequence
  Adh900 split marker cassette 1
cactccagttgggccattaccgaacattttgccattgtaggcgattagtaagtattaacaagacagctgactatacgtttattctcaaacaatatttccctttttggttttgacctcgctttaatcaatttttcagacctgatcccacctacttttcttcggcctcaacttcaatctgactcttctctctcaattggtaccaaccagccagaaaatgtccttccgttacttgaaacggcatttctctacagctacaaacgcaattgctctccttagcagacctgaattcaaaataggtcgaattgtggacgtcgtgaaacatccaaatgcagacaaactttatgtctcgtcgatttctgtgggaaacaattatgcctcgggtacatccaacaccctaaccgtttgcagcggcttggtggactacttttcagttcccgaattgcttcagcgacgggtcgttgtggtcacaaacctcaagccatcgaagatgagaggtgtaacatcggaggcaatgcttttggcaggggaaaagtcggggaaagtggaattggtcgagccgccaatgtccgggagagagggcgaatcactccacttcgaaggtgtagaaattacatcagaggagagcgccaatcaattgcatttgcctgctaagcgattgaagaagtcagagtggagtcaactggcggaaggtctacagacaaatgaccagcgtgaagtggtcttccacagccaaattggctccaaacgaatttacgctttagtaggagcgagtactgaaaaatgcacgttagcgactcttgcgcaggccgtcgtacgataagggcaatatggttgagaacgttcctcacccaaataaaatcatcgtacgctgcaggtcgacaacccttaatataacttcgtataatgtatgctatacgaagttattaggtctagatcggtaccgacatggaggcccagaataccctccttgacagtcttgacgtgcgcagctcaggggcatgatgtgactgtcgcccgtacatttagcccatacatccccatgtataatcatttgcatccatacattttgatggccgcacggcgcgaagcaaaaattacggctcctcgctgcagacctgcgagcagggaaacgctcccctcacagacgcgttgaattgtccccacgccgcgcccctgtagagaaatataaaaggttaggatttgccactgaggttcttctttcatatacttccttttaaaatcttgctaggatacagttctcacatcacatccgaacataaacaaccatgggtaaggaaaagactcacgtttcgaggccgcgattaaattccaacatggatgctgatttatatgggtataaatgggctcgcgataatgtcgggcaatcaggtgcgacaatctatcgattgtatgggaagcccgatgcgccagagttgtttctgaaacatggcaaaggtagcgttgccaatgatgttacagatgagatggtcagactaaactggctgacggaatttatgcctcttccgaccatcaagcattttatccgtactcctgatgatgcatggttactcaccactgcgatccccggcaaaacagcattccaggtattagaagaatatcctgattcaggtgaaaatattgttgatgcgctggcagtgttcctgcgccggttgcattcgattcctgtttgtaattgtccttttaacagcgatcgcgtatttcgtctcgctcaggcgcaatcacgaatgaataacggtttggttgatgcgagtgattttgatgacgagcgtaatggctggcctgttgaacaagtctggaaagaaatgcataagcttttgccattctcaccg

SEQ ID NO: 75 - DNA, 1993 bp, Artificial Sequence
  Adh900 split marker cassette 2
aagcccgatgcgccagagttgtttctgaaacatggcaaaggtagcgttgccaatgatgttacagatgagatggtcagactaaactggctgacggaatttatgcctcttccgaccatcaagcattttatccgtactcctgatgatgcatggttactcaccactgcgatccccggcaaaacagcattccaggtattagaagaatatcctgattcaggtgaaaatattgttgatgcgctggcagtgttcctgcgccggttgcattcgattcctgtttgtaattgtccttttaacagcgatcgcgtatttcgtctcgctcaggcgcaatcacgaatgaataacggtttggttgatgcgagtgattttgatgacgagcgtaatggctggcctgttgaacaagtctggaaagaaatgcataagcttttgccattctcaccggattcagtcgtcactcatggtgatttctcacttgataaccttatttttgacgaggggaaattaataggttgtattgatgttggacgagtcggaatcgcagaccgataccaggatcttgccatcctatggaactgcctcggtgagttttctccttcattacagaaacggctttttcaaaaatatggtattgataatcctgatatgaataaattgcagtttcatttgatgctcgatgagtttttctaatcagtactgacaataaaaagattcttgttttcaagaacttgtcatttgtatagtttttttatattgtagttgttctattttaatcaaatgttagcgtgatttatattttttttcgcctcgacatcatctgcccagatgcgaagttaagtgcgcagaaagtaatatcatgcgtcaatcgtatgtgaatgctggtcgctatactggtaccattcgagaacccttaatataacttcgtataatgtatgctatacgaagttattaggtgatatcagatccactctgtagtgagggttggtggtctgacgaacatccagcaaggtgttccacctgaaatttttcaccttggagggtaatgtgatgacgccatttcctgtgcaaatgcttttcgttttgaacagtgcaacttttgtatcagatcttcatctacttgatgccatctcaacaaatccctcatttactagcgtgtgaaggaatctagattttccactgataagccaatttgtcggaaatcccccgcgcgggagttggcgttcagtacgagccacacacgtttcttttggacaaccaaagcatccgcctgaagggacaacttgcattcaacggcttcagttggaaacgtcagagctgacctatagtttgctagaaccgttttctctgtttacgtttacgtctcctcaaatttgcgctcggtatgtccttcctaattagcgggaaaagctgttcttagttaatacggagaaagtttcggggttaccgttccgggaagaggaggggtcatctctctcatctcatccaaccattaagtttcttccaaaacttcaggataatcagtttaaccaccgacaggagtcagatttgagattgacagaaagtttttccgtccatttcctcatcttgtcgccgttatcagtcaatctctatggttatctggaatttcttttttcttttaattcatcttctttttatcccgcgcctttggcgttctagctcatctcatgaaaacaaaaccctctcatgttcggataattccagcggctttcactttcagatgacacatagattggactcaaccatggctatctggggtatacggacgttggcaagggcgttaatttttcaggacaaacggaaatgccatggctccagggaaaggcattcctattgcaaacctagaccgtcgaacctctcctatcgcctaccagtcacccagctatccctaggcaactcatctccttcaagcggattgcaacctgctaagccaaattagatctggccacagaaatgccgcaatatttcttggctctcccctccc

SEQ ID NO: 76 - DNA, 23 bp, Artificial Sequence
  Primer sequence
gaattgagccaaaaaaggagagg

SEQ ID NO: 77 - DNA, 23 bp, Artificial Sequence
  Primer sequence
gatggaataggagactaggtgtg

SEQ ID NO: 78 - DNA, 20 bp, Artificial Sequence
  Primer sequence
tggttgagacgtttgtattg

SEQ ID NO: 79 - DNA, 18 bp, Artificial Sequence
  Primer sequence
tgggttgggagtttagtg

SEQ ID NO: 80 - DNA, 1053 bp, Artificial Sequence; identical to SEQ ID NO: 51
  ADH2 coding sequence

SEQ ID NO: 81 - DNA, 1083 bp, Artificial Sequence
  ADH900 coding sequence
atgtctgtgatgaaagccctcgtgtacggtggtaagaacgtcttcgcctggaaaaacttccctaaaccaactatcttgcacccaacagatgtcatcgttaagacggtggctactaccatctgcggaacagacttgcacatcttgaaaggtgatgttccagaggtcaaacctgaaaccgtcttgggtcatgaagcaattggagtcgtcgaatctatcggtgataacgtcaaaaacttcagcattggtgataaggtgctggtttcatgcatcaccagttgtggaagctgttactactgtaagagaaacttgcagagtcattgcaagaccggtggatggaaattaggtcacgatttgaacggtacgcaggctgagtttgtccgtatcccatatggagacttctcattgcaccgtattcctcatgaagcagatgaaaaggcagttctgatgctgtctgacatcttacctactgcttacgaagttggtgttcttgccggaaatgtccaaaagggagactcagttgccattgtcggcgccggtccagttggtcttgccgctctgctgactgtcaaagcctttgagccttctgaaattattatgattgacactaacgatgaaagactgagtgcctccttgaaattgggagccaccaaggcagtcaacccaaccaaggtcagcagtgtcaaagatgctgtttatgatattgtcaatgccactgtccgcgtcaaggagaacgacctggagccaggtgtcgatgttgccattgagtgtgttggtgttcctgacacgtttgcaacttgtgaagagattatcgccccaggtggccgtattgccaatgttggtgttcacggcactaaagtggatttacaactgcaagacctatggatcaagaacattgctatcaccaccggtttggtagccacatactccactaaagacctgttgaagcgagtctctgacaagtctctagaccctacaccactggttacacatgagttcaagttcagtgaatttgagaaggcctatgagacttctcaaaatgctgccaccaccaaagccatcaagattttcttatctgccgattaa

SEQ ID NO: 82 - DNA, 1080 bp, Artificial Sequence
  Adh2_GG_cured
gataggtctcacatgtctccaactatcccaactacacaaaaggctgttatcttcgaaaccaacggcggtcccctagagtacaaggacattccagtcccaaagccaaagtcaaacgaacttttgatcaacgttaagtactccggtgtctgtcacactgatttgcacgcctggaagggtgactggccattggacaacaagcttcctttggttggtggtcacgaaggtgctggtgtcgttgtcgcttacggtgagaacgtcactggatgggagatcggtgactacgctggtatcaaatggttgaacggttcttgtttgaactgtgagtactgtatccaaggtgctgaatccagttgtgccaaggctgacctgtctggtttcacccacgacggatctttccagcagtatgctactgctgatgccacccaagccgccagaattccaaaggaggctgacttggctgaagttgccccaattctgtgtgctggtatcaccgtttacaaggctcttaagaccgctgacttgcgtattggccaatgggttgccatttctggtgctggtggaggactgggttctcttgccgttcaatacgccaaggctctgggtttgagagttttgggtattgatggtggtgccgacaagggtgaatttgtcaagtccttgggtgctgaggtgttcgtcgacttcactaagactaaggacgtcgttgctgaagtccaaaagctcaccaacggtggtccacacggtgttattaacgtctccgtttccccacatgctatcaaccaatctgtccaatacgttagaactttgggtaaggttgttttggttggtctgccatctggtgccgttgtcaactctgacgttttctggcacgttctgaagtccatcgagatcaagggatcttacgttggaaacagagaggacagtgccgaggccatcgacttgttcaccagaggtttggtcaaggctcctatcaagattatcggtctgtctgaacttgctaaggtctacgaacagatggaggctggtgccatcatcggtagatacgttgtggacacttccaaataagcttagagaccgatc

SEQ ID NO: 83 - DNA, 1110 bp, Artificial Sequence
  Adh900_GG_cured
gataggtctcacatgtctgtgatgaaagccctcgtgtacggtggtaagaacgtgttcgcctggaaaaacttccctaaaccaactatcttgcacccaacagatgtcatcgttaagacggtggctactaccatctgcggaacagacttgcacatcttgaaaggtgatgttccagaggtcaaacctgaaaccgtcttgggtcatgaagcaattggagtcgtcgaatctatcggtgataacgtcaaaaacttcagcattggtgataaggtgctggtttcatgcatcaccagttgtggaagctgttactactgtaagagaaacttgcagagtcattgcaagaccggtggatggaaattaggtcacgatttgaacggtacgcaggctgagtttgtccgtatcccatatggagacttctcattgcaccgtattcctcatgaagcagatgaaaaggcagttctgatgctgtctgacatcttacctactgcttacgaagttggtgttcttgccggaaatgtccaaaagggagactcagttgccattgtcggcgccggtccagttggtcttgccgctctgctgactgtcaaagcctttgagccttctgaaattattatgattgacactaacgatgaaagactgagtgcctccttgaaattgggagccaccaaggcagtcaacccaaccaaggtcagcagtgtcaaagatgctgtttatgatattgtcaatgccactgtccgcgtcaaggagaacgacctggagccaggtgtcgatgttgccattgagtgtgttggtgttcctgacacgtttgcaacttgtgaagagattatcgccccaggtggccgtattgccaatgttggtgttcacggcactaaagtggatttacaactgcaagacctatggatcaagaacattgctatcaccaccggtttggtagccacatactccactaaagacctgttgaagcgagtctctgacaagtctctagaccctacaccactggttacacatgagttcaagttcagtgaatttgagaaggcctatgagacttctcaaaatgctgccaccaccaaagccatcaagattttcttatctgccgattaagcttagagaccgatc

SEQ ID NO: 84 - DNA, 21 bp, Artificial Sequence
  Primer sequence
ttgatcttttctacggggtgg

SEQ ID NO: 85 - DNA, 20 bp, Artificial Sequence
  Primer sequence
ggtgttttgaagtggtacgg